European Patent Application EP 4 212 544 A1, published July 19, 2023. Title: A Receptor Binding Domain variants of Coronavirus with reduced ACE2 binding affinity and Vaccine composition comprising the same. Applicant: GI Cell, Inc. The sequence listing filed with the application follows.

SEQUENCE LISTING (82 sequences)

SEQ ID NO: 1 - protein, 219 aa, Artificial Sequence
  Wild type RBD
RVQPTESIVRFPNITNLCPFGEVFNATRFASVYAWNRKRISNCVADYSVLYNSASFSTFKCYGVSPTKLNDLCFTNVYADSFVIRGDEVRQIAPGQTGKIADYNYKLPDDFTGCVIAWNSNNLDSKVGGNYNYLYRLFRKSNLKPFERDISTEIYQAGSTPCNGVEGFNCYFPLQSYGFQPTNGVGYQPYRVVVLSFELLHAPATVCGPKKSTNLVKNK

SEQ ID NO: 2 - protein, 231 aa, Artificial Sequence
  IgG1 Fc domain
EPKSSDKTHTCPPCPAPELLGGPSVFLFPPKPKDTLMISRTPEVTCVVVDVSHEDPEVKFNWYVDGVEVHNAKTKPREEQYNSTYRVVSVLTVLHQDWLNGKEYKCKVSNKALPAPIEKTISKAKGQPREPQVYTLPPSRDELTKNQVSLTCLVKGFYPSDIAVEWESNGQPENNYKTTPPVLDSDGSFFLYSKLTVDKSRWQQGNVFSCSVMHEALHNHYTQKSLSLSPG

SEQ ID NO: 3 - protein, 419 aa, Artificial Sequence
  N protein_full
MSDNGPQNQRNAPRITFGGPSDSTGSNQNGERSGARSKQRRPQGLPNNTASWFTALTQHGKEDLKFPRGQGVPINTNSSPDDQIGYYRRATRRIRGGDGKMKDLSPRWYFYYLGTGPEAGLPYGANKDGIIWVATEGALNTPKDHIGTRNPANNAAIVLQLPQGTTLPKGFYAEGSRGGSQASSRSSSRSRNSSRNSTPGSSRGTSPARMAGNGGDAALALLLLDRLNQLESKMSGKGQQQQGQTVTKKSAAEASKKPRQKRTATKAYNVTQAFGRRGPEQTQGNFGDQELIRQGTDYKHWPQIAQFAPSASAFFGMSRIGMEVTPSGTWLTYTGAIKLDDKDPNFKDQVILLNKHIDAYKTFPPTEPKKDKKKKADETQALPQRQKKQQTVTLLPAADLDDFSKQLQQSMSSADSTQA

SEQ ID NO: 4 - protein, 156 aa, Artificial Sequence
  N protein_RNA binding domain
RSKQRRPQGLPNNTASWFTALTQHGKEDLKFPRGQGVPINTNSSPDDQIGYYRRATRRIRGGDGKMKDLSPRWYFYYLGTGPEAGLPYGANKDGIIWVATEGALNTPKDHIGTRNPANNAAIVLQLPQGTTLPKGFYAEGSRGGSQASSRSSSRSR

SEQ ID NO: 5 - protein, 122 aa, Artificial Sequence
  M protein
RLFARTRSMWSFNPETNILLNVPLHGTILTRPLLESELVIGAVILRGHLRIAGHHLGRCDIKDLPKEITVATSRTLSYYKLGASQRVAGDSGFAAYSRYRIGNYKLNTDHSSSSDNIALLVQ

SEQ ID NO: 6 - protein, 15 aa, Artificial Sequence
  Linker1
GGGGSGGGGSGGGGS

SEQ ID NO: 7 - protein, 20 aa, Artificial Sequence
  Linker2
GGGGSGGGGSGGGGSGGGGS

SEQ ID NO: 8 - protein, 10 aa, Artificial Sequence
  Linker3
GGGGSGGGGS

SEQ ID NO: 9 - protein, 9 aa, Artificial Sequence
  Linker4
GGSGGSGGS

SEQ ID NO: 10 - protein, 12 aa, Artificial Sequence
  Linker5
GGSGGSGGSGGS

SEQ ID NO: 11 - protein, 9 aa, Artificial Sequence
  Linker6
GGSGGSGGS

SEQ ID NO: 12 - protein, 18 aa, Artificial Sequence
  Signal peptide
MKWVTFISLLFLFSSAYS

SEQ ID NO: 13 - protein, 219 aa, Artificial Sequence
  RBDm(Q175A, N183A)
RVQPTESIVRFPNITNLCPFGEVFNATRFASVYAWNRKRISNCVADYSVLYNSASFSTFKCYGVSPTKLNDLCFTNVYADSFVIRGDEVRQIAPGQTGKIADYNYKLPDDFTGCVIAWNSNNLDSKVGGNYNYLYRLFRKSNLKPFERDISTEIYQAGSTPCNGVEGFNCYFPLASYGFQPTAGVGYQPYRVVVLSFELLHAPATVCGPKKSTNLVKNK

SEQ ID NO: 14 - protein, 219 aa, Artificial Sequence
  RBDm(G164A, V165A, Q175A, S176A, N183A)
RVQPTESIVRFPNITNLCPFGEVFNATRFASVYAWNRKRISNCVADYSVLYNSASFSTFKCYGVSPTKLNDLCFTNVYADSFVIRGDEVRQIAPGQTGKIADYNYKLPDDFTGCVIAWNSNNLDSKVGGNYNYLYRLFRKSNLKPFERDISTEIYQAGSTPCNAAEGFNCYFPLAAYGFQPTAGVGYQPYRVVVLSFELLHAPATVCGPKKSTNLVKNK

SEQ ID NO: 15 - protein, 219 aa, Artificial Sequence
  RBDm(L137A, G164A, V165A, F168A, Q175A, S176A, N183A)
RVQPTESIVRFPNITNLCPFGEVFNATRFASVYAWNRKRISNCVADYSVLYNSASFSTFKCYGVSPTKLNDLCFTNVYADSFVIRGDEVRQIAPGQTGKIADYNYKLPDDFTGCVIAWNSNNLDSKVGGNYNYLYRAFRKSNLKPFERDISTEIYQAGSTPCNAAEGANCYFPLAAYGFQPTAGVGYQPYRVVVLSFELLHAPATVCGPKKSTNLVKNK

SEQ ID NO: 16 - protein, 219 aa, Artificial Sequence
  RBDm(L137A, F168A)
RVQPTESIVRFPNITNLCPFGEVFNATRFASVYAWNRKRISNCVADYSVLYNSASFSTFKCYGVSPTKLNDLCFTNVYADSFVIRGDEVRQIAPGQTGKIADYNYKLPDDFTGCVIAWNSNNLDSKVGGNYNYLYRAFRKSNLKPFERDISTEIYQAGSTPCNGVEGANCYFPLQSYGFQPTNGVGYQPYRVVVLSFELLHAPATVCGPKKSTNLVKNK

SEQ ID NO: 17 - protein, 219 aa, Artificial Sequence
  RBDm(L137A)
RVQPTESIVRFPNITNLCPFGEVFNATRFASVYAWNRKRISNCVADYSVLYNSASFSTFKCYGVSPTKLNDLCFTNVYADSFVIRGDEVRQIAPGQTGKIADYNYKLPDDFTGCVIAWNSNNLDSKVGGNYNYLYRAFRKSNLKPFERDISTEIYQAGSTPCNGVEGFNCYFPLQSYGFQPTNGVGYQPYRVVVLSFELLHAPATVCGPKKSTNLVKNK

SEQ ID NO: 18 - protein, 219 aa, Artificial Sequence
  RBDm(F168A)
RVQPTESIVRFPNITNLCPFGEVFNATRFASVYAWNRKRISNCVADYSVLYNSASFSTFKCYGVSPTKLNDLCFTNVYADSFVIRGDEVRQIAPGQTGKIADYNYKLPDDFTGCVIAWNSNNLDSKVGGNYNYLYRLFRKSNLKPFERDISTEIYQAGSTPCNGVEGANCYFPLQSYGFQPTNGVGYQPYRVVVLSFELLHAPATVCGPKKSTNLVKNK

SEQ ID NO: 19 - protein, 219 aa, Artificial Sequence
  RBDm(G184D)
RVQPTESIVRFPNITNLCPFGEVFNATRFASVYAWNRKRISNCVADYSVLYNSASFSTFKCYGVSPTKLNDLCFTNVYADSFVIRGDEVRQIAPGQTGKIADYNYKLPDDFTGCVIAWNSNNLDSKVGGNYNYLYRLFRKSNLKPFERDISTEIYQAGSTPCNGVEGFNCYFPLQSYGFQPTNDVGYQPYRVVVLSFELLHAPATVCGPKKSTNLVKNK

SEQ ID NO: 20 - DNA, 657 bp, Artificial Sequence
  Wild type RBD_DNA sequence
agagttcagcctaccgagtccatcgtgcggttccccaacatcaccaacctgtgtcctttcggcgaggtgttcaacgctaccagattcgcctctgtgtacgcctggaaccggaagcggatctctaactgcgtggccgactactccgtgctgtacaactctgcctccttcagcaccttcaagtgctacggcgtgtcccctaccaagctgaacgacctgtgcttcaccaacgtgtacgccgactccttcgtgatcaggggcgacgaagttcggcagatcgctcctggacagaccggcaagatcgccgactacaattacaagctgcccgacgacttcaccggctgcgtgatcgcttggaactccaacaacctggactccaaagtcggcggcaactacaactacctgtaccggctgttccggaagtccaacctgaagcctttcgagcgggacatctccaccgagatctaccaggctggcagcaccccttgcaatggcgtcgagggcttcaactgctacttcccactgcagtcctacggcttccagcctaccaatggcgtgggctaccagccttatagagtggtggtgctgtccttcgagctgctgcatgctcctgctaccgtgtgcggccctaagaaatctaccaacctggtcaagaacaag

SEQ ID NO: 21 - DNA, 693 bp, Artificial Sequence
  IgG1 Fc domain-DNA sequence
gaacctaagtcctccgacaagacccacacctgtcctccatgtcctgctccagaactgctcggcggaccttccgtgtttctgttcccacctaagccaaaggacaccctgatgatcagcagaacccctgaagtgacctgcgtggtggtggatgtgtctcacgaggaccccgaagtgaagttcaattggtacgtggacggcgtggaagtgcacaacgccaagaccaagcctagagaggaacagtacaactccacctacagagtggtgtccgtgctgaccgtgctgcaccaggattggctgaacggcaaagagtacaagtgcaaggtgtccaacaaggccctgcctgctcctatcgaaaagaccatctccaaggccaagggccagcctagggaaccccaggtttacacactgcctccatctcgggacgagctgaccaagaatcaggtgtccctgacctgtctggtcaagggcttctacccttccgatatcgccgtggaatgggagagcaatggccagcctgagaacaactacaagacaacccctcctgtgctggactccgacggctcattcttcctgtatagcaagctgacagtggacaagtcccggtggcagcagggcaacgtgttctcctgttctgtgatgcacgaggccctgcacaaccactacacccagaagagtctgtccttgagcccgggc

SEQ ID NO: 22 - DNA, 1260 bp, Artificial Sequence
  N protein_full DNA sequence
atgtctgataatggaccccaaaatcagcgaaatgcaccccgcattacgtttggtggaccctcagattcaactggcagtaaccagaatggagaacgcagtggggcgcgatcaaaacaacgtcggccccaaggtttacccaataatactgcgtcttggttcaccgctctcactcaacatggcaaggaagaccttaaattccctcgaggacaaggcgttccaattaacaccaatagcagtccagatgaccaaattggctactaccgaagagctaccagacgaattcgtggtggtgacggtaaaatgaaagatctcagtccaagatggtatttctactacctaggaactgggccagaagctggacttccctatggtgctaacaaagacggcatcatatgggttgcaactgagggagccttgaatacaccaaaagatcacattggcacccgcaatcctgctaacaatgctgcaatcgtgctacaacttcctcaaggaacaacattgccaaaaggcttctacgcagaagggagcagaggcggcagtcaagcctcttctcgttcctcatcacgtagtcgcaacagttcaagaaattcaactccaggcagcagtaggggaacttctcctgctagaatggctggcaatggcggtgatgctgctcttgctttgctgctgcttgacagattgaaccagcttgagagcaaaatgtctggtaaaggccaacaacaacaaggccaaactgtcactaagaaatctgctgctgaggcttctaagaagcctcggcaaaaacgtactgccactaaagcatacaatgtaacacaagctttcggcagacgtggtccagaacaaacccaaggaaattttggggaccaggaactaatcagacaaggaactgattacaaacattggccgcaaattgcacaatttgcccccagcgcttcagcgttcttcggaatgtcgcgcattggcatggaagtcacaccttcgggaacgtggttgacctacacaggtgccatcaaattggatgacaaagatccaaatttcaaagatcaagtcattttgctgaataagcatattgacgcatacaaaacattcccaccaacagagcctaaaaaggacaaaaagaagaaggctgatgaaactcaagccttaccgcagagacagaagaaacagcaaactgtgactcttcttcctgctgcagatttggatgatttctccaaacaattgcaacaatccatgagcagtgctgactcaactcaggcctaa

SEQ ID NO: 23 - DNA, 468 bp, Artificial Sequence
  N protein_RNA binding domain_DNA sequence
cggtctaagcagagaaggcctcagggcctgcctaacaataccgcctcctggtttaccgctctgacccagcacggcaaagaggacctgaagttccctagaggacagggcgtgcccatcaacaccaactctagccctgacgaccagatcggctactacagacgggccaccagaagaatcagaggcggcgacggcaagatgaaggacctgtctcctcggtggtacttctactacctcggcaccggaccagaggctggattgccttatggcgccaacaaggacggcatcatctgggttgcaacagagggcgctctgaacacccctaaggaccacatcggcacccggaatcctgccaacaatgctgccattgtgctgcagctgccacagggcacaacactgcctaagggcttttacgccgagggctctagaggcggctctcaggcctcttccagatcctccagtagatcacgt

SEQ ID NO: 24 - DNA, 366 bp, Artificial Sequence
  M protein_DNA sequence
cggctgttcgcccggaccagatctatgtggtctttcaaccccgagacaaacatcctgctgaacgtgccactgcacggcaccatcctgaccagacctctgctggaatccgagctggtcatcggcgctgtgatcctgagaggccacctgagaatcgctggccaccatctgggcagatgcgacatcaaggacctgcctaaagagatcaccgtcgccacctctcggaccctgagctactataagctgggcgcctctcagagagtggctggcgattctggctttgccgcctactccagataccggatcggcaactacaagctgaacaccgaccactcctccagctccgacaatatcgctctgctggtgcag

SEQ ID NO: 25 - DNA, 45 bp, Artificial Sequence
  Linker1_DNA sequence
ggcggcggaggatccggcggtggtggttccggcggaggcggttct

SEQ ID NO: 26 - DNA, 60 bp, Artificial Sequence
  Linker2_DNA sequence
ggtggcggcggttcaggcggcggtggaagtggcggtggcggatctggcggaggtggtagt

SEQ ID NO: 27 - DNA, 30 bp, Artificial Sequence
  Linker3_DNA sequence
ggcggaggcggatctggtggcggaggatct

SEQ ID NO: 28 - DNA, 27 bp, Artificial Sequence
  Linker4_DNA sequence
ggtggcagtggtggctctggcggatct

SEQ ID NO: 29 - DNA, 36 bp, Artificial Sequence
  Linker5_DNA sequence
ggcggatccggaggatcaggtggaagcggaggttca

SEQ ID NO: 30 - DNA, 27 bp, Artificial Sequence
  Linker6_DNA sequence
ggtggtagtggcggaagcggcggctcc

SEQ ID NO: 31 - DNA, 54 bp, Artificial Sequence
  Signal peptide_DNA sequence
atgaaatgggtcacctttatctccctgctgttcctgttctcctccgcctactct

SEQ ID NO: 32 - DNA, 657 bp, Artificial Sequence
  RBDm(Q175A, N183A)_DNA sequece
agagtgcagcctaccgagtctatcgtgcggttccccaacatcaccaacctgtgtcctttcggcgaggtgttcaacgccaccagattcgcctctgtgtacgcctggaaccggaagcggatctctaactgcgtggccgactactccgtgctgtacaactccgcctccttcagcaccttcaagtgctacggcgtgtcccctaccaagctgaacgacctgtgcttcaccaacgtgtacgccgactccttcgtgatcagaggcgacgaagtgcggcagatcgctcctggacagaccggcaagatcgccgactacaactacaagctgcccgacgacttcaccggctgtgtgatcgcttggaactccaacaacctggactccaaagtcggcggcaactacaattacctgtaccggctgttccggaagtccaacctgaagcctttcgagcgggacatctccaccgagatctaccaggctggcagcaccccttgtaatggcgtggaaggcttcaactgctacttccctctggcctcctacggcttccaacctacagctggcgtgggctaccagccttacagagtggtggtgctgtccttcgagctgctgcatgctcctgctaccgtgtgcggccctaagaaatctaccaacctggtcaagaacaag

SEQ ID NO: 33 - DNA, 657 bp, Artificial Sequence
  RBDm(G164A, V165A, Q175A, S176A, N183A)_DNA sequece
agagtgcagcctaccgagtctatcgtgcggttccccaacatcaccaacctgtgtcctttcggcgaggtgttcaacgccaccagattcgcctctgtgtacgcctggaaccggaagcggatctctaactgcgtggccgactactccgtgctgtacaactccgcctccttcagcaccttcaagtgctacggcgtgtcccctaccaagctgaacgacctgtgcttcaccaacgtgtacgccgactccttcgtgatcagaggcgacgaagtgcggcagatcgctcctggacagaccggcaagatcgccgactacaactacaagctgcccgacgacttcaccggctgtgtgatcgcttggaactccaacaacctggactccaaagtcggcggcaactacaattacctgtaccggctgttccggaagtccaacctgaagcctttcgagcgggacatctccaccgagatctaccaggctggcagcaccccttgtaatgccgccgagggcttcaactgctactttcctctggccgcctacggcttccaacctacagctggcgttggctaccagccttacagagtggtggtgctgtccttcgagctgctgcatgctcctgctaccgtgtgcggccctaagaaatctaccaacctggtcaagaacaag

SEQ ID NO: 34 - DNA, 657 bp, Artificial Sequence
  RBDm(L137A, G164A, V165A, F168A, Q175A, S176A, N183A)_DNA sequece
agagtgcagcctaccgagtctatcgtgcggttccccaacatcaccaacctgtgtcctttcggcgaggtgttcaacgccaccagattcgcctctgtgtacgcctggaaccggaagcggatctctaactgcgtggccgactactccgtgctgtacaactccgcctccttcagcaccttcaagtgctacggcgtgtcccctaccaagctgaacgacctgtgcttcaccaacgtgtacgccgactccttcgtgatcagaggcgacgaagtgcggcagatcgctcctggacagaccggcaagatcgccgactacaactacaagctgcccgacgacttcaccggctgtgtgatcgcttggaactccaacaacctggactccaaagtcggcggcaactacaattacctgtaccgggccttccgcaagtccaacctgaagcctttcgagcgggacatctccaccgagatctaccaggctggcagcaccccttgtaatgctgccgaaggcgccaactgctactttcctctggccgcctatggcttccagcctacagctggcgttggctaccagccttatagagtggtggtgctgtccttcgagctgctgcatgctcctgctaccgtgtgcggccctaagaaatctaccaacctggtcaagaacaaa

SEQ ID NO: 35 - DNA, 657 bp, Artificial Sequence
  RBDm(L137A, F168A)_DNA sequece
agagtgcagcctaccgagtccatcgtgcggttccccaacatcaccaacctgtgtcctttcggcgaggtgttcaacgctaccagattcgcctctgtgtacgcctggaaccggaagcggatctctaactgcgtggccgactactccgtgctgtacaactctgcctccttcagcaccttcaagtgctacggcgtgtcccctaccaagctgaacgacctgtgcttcaccaacgtgtacgccgactccttcgtgatcaggggcgacgaagttcggcagatcgctcctggacagaccggcaagatcgccgactacaattacaagctgcccgacgacttcaccggctgcgtgatcgcttggaactccaacaacctggactccaaagtcggcggcaactacaactacctgtaccgggccttcagaaagtccaacctgaagcctttcgagcgggacatctccaccgagatctaccaggctggcagcaccccttgcaatggcgttgaaggcgccaactgctacttcccactgcagtcctacggcttccagcctaccaatggcgtgggctaccagccttatagagtggtggtgctgtccttcgagctgctgcatgctcctgctacagtgtgcggccccaagaaatctaccaacctggtcaagaacaag

SEQ ID NO: 36 - DNA, 657 bp, Artificial Sequence
  RBDm(L137A)_DNA sequece
agagtgcagcctaccgagtccatcgtgcggttccccaacatcaccaacctgtgtcctttcggcgaggtgttcaacgctaccagattcgcctctgtgtacgcctggaaccggaagcggatctctaactgcgtggccgactactccgtgctgtacaactctgcctccttcagcaccttcaagtgctacggcgtgtcccctaccaagctgaacgacctgtgcttcaccaacgtgtacgccgactccttcgtgatcaggggcgacgaagttcggcagatcgctcctggacagaccggcaagatcgccgactacaattacaagctgcccgacgacttcaccggctgcgtgatcgcttggaactccaacaacctggactccaaagtcggcggcaactacaactacctgtaccgggccttcagaaagtccaacctgaagcctttcgagcgggacatctccaccgagatctaccaggctggcagcaccccttgcaatggcgttgaaggcttcaactgctacttcccactgcagtcctacggcttccagcctaccaatggcgtgggctaccagccttatagagtggtggtgctgtccttcgagctgctgcatgctcctgctacagtgtgcggccccaagaaatctaccaacctggtcaagaacaag

SEQ ID NO: 37 - DNA, 657 bp, Artificial Sequence
  RBDm(F168A)_DNA sequece
agagtgcagcctaccgagtccatcgtgcggttccccaacatcaccaacctgtgtcctttcggcgaggtgttcaacgctaccagattcgcctctgtgtacgcctggaaccggaagcggatctctaactgcgtggccgactactccgtgctgtacaactctgcctccttcagcaccttcaagtgctacggcgtgtcccctaccaagctgaacgacctgtgcttcaccaacgtgtacgccgactccttcgtgatcaggggcgacgaagttcggcagatcgctcctggacagaccggcaagatcgccgactacaattacaagctgcccgacgacttcaccggctgcgtgatcgcttggaactccaacaacctggactccaaagtcggcggcaactacaactacctgtaccggctgttcagaaagtccaacctgaagcctttcgagcgggacatctccaccgagatctaccaggctggcagcaccccttgcaatggcgttgaaggcgccaactgctacttcccactgcagtcctacggcttccagcctaccaatggcgtgggctaccagccttatagagtggtggtgctgtccttcgagctgctgcatgctcctgctacagtgtgcggccccaagaaatctaccaacctggtcaagaacaag

SEQ ID NO: 38 - DNA, 657 bp, Artificial Sequence
  RBDm(G184D)_DNA sequence
agagttcagcctaccgagtccatcgtgcggttccccaacatcaccaacctgtgtcctttcggcgaggtgttcaacgctaccagattcgcctctgtgtacgcctggaaccggaagcggatctctaactgcgtggccgactactccgtgctgtacaactctgcctccttcagcaccttcaagtgctacggcgtgtcccctaccaagctgaacgacctgtgcttcaccaacgtgtacgccgactccttcgtgatcaggggcgacgaagttcggcagatcgctcctggacagaccggcaagatcgccgactacaattacaagctgcccgacgacttcaccggctgcgtgatcgcttggaactccaacaacctggactccaaagtcggcggcaactacaactacctgtaccggctgttccggaagtccaacctgaagcctttcgagcgggacatctccaccgagatctaccaggctggcagcaccccttgcaatggcgtcgagggcttcaactgctacttcccactgcagtcctacggcttccagcctaccaatgacgtgggctaccagccttatagagtggtggtgctgtccttcgagctgctgcatgctcctgctaccgtgtgcggccctaagaaatctaccaacctggtcaagaacaag

SEQ ID NO: 39 - protein, 246 aa, Artificial Sequence
  Fusion protein_IgG1 Fc
GGGGSGGGGSGGGGSEPKSSDKTHTCPPCPAPELLGGPSVFLFPPKPKDTLMISRTPEVTCVVVDVSHEDPEVKFNWYVDGVEVHNAKTKPREEQYNSTYRVVSVLTVLHQDWLNGKEYKCKVSNKALPAPIEKTISKAKGQPREPQVYTLPPSRDELTKNQVSLTCLVKGFYPSDIAVEWESNGQPENNYKTTPPVLDSDGSFFLYSKLTVDKSRWQQGNVFSCSVMHEALHNHYTQKSLSLSPG

SEQ ID NO: 40 - protein, 465 aa, Artificial Sequence
  Fusion protein_RBDwt-Fc
RVQPTESIVRFPNITNLCPFGEVFNATRFASVYAWNRKRISNCVADYSVLYNSASFSTFKCYGVSPTKLNDLCFTNVYADSFVIRGDEVRQIAPGQTGKIADYNYKLPDDFTGCVIAWNSNNLDSKVGGNYNYLYRLFRKSNLKPFERDISTEIYQAGSTPCNGVEGFNCYFPLQSYGFQPTNGVGYQPYRVVVLSFELLHAPATVCGPKKSTNLVKNKGGGGSGGGGSGGGGSEPKSSDKTHTCPPCPAPELLGGPSVFLFPPKPKDTLMISRTPEVTCVVVDVSHEDPEVKFNWYVDGVEVHNAKTKPREEQYNSTYRVVSVLTVLHQDWLNGKEYKCKVSNKALPAPIEKTISKAKGQPREPQVYTLPPSRDELTKNQVSLTCLVKGFYPSDIAVEWESNGQPENNYKTTPPVLDSDGSFFLYSKLTVDKSRWQQGNVFSCSVMHEALHNHYTQKSLSLSPG

SEQ ID NO: 41 - protein, 485 aa, Artificial Sequence
  Fusion protein_Fc-RBDwt
GGGGSGGGGSGGGGSEPKSSDKTHTCPPCPAPELLGGPSVFLFPPKPKDTLMISRTPEVTCVVVDVSHEDPEVKFNWYVDGVEVHNAKTKPREEQYNSTYRVVSVLTVLHQDWLNGKEYKCKVSNKALPAPIEKTISKAKGQPREPQVYTLPPSRDELTKNQVSLTCLVKGFYPSDIAVEWESNGQPENNYKTTPPVLDSDGSFFLYSKLTVDKSRWQQGNVFSCSVMHEALHNHYTQKSLSLSPGGGGGSGGGGSGGGGSGGGGSRVQPTESIVRFPNITNLCPFGEVFNATRFASVYAWNRKRISNCVADYSVLYNSASFSTFKCYGVSPTKLNDLCFTNVYADSFVIRGDEVRQIAPGQTGKIADYNYKLPDDFTGCVIAWNSNNLDSKVGGNYNYLYRLFRKSNLKPFERDISTEIYQAGSTPCNGVEGFNCYFPLQSYGFQPTNGVGYQPYRVVVLSFELLHAPATVCGPKKSTNLVKNK

SEQ ID NO: 42 - protein, 402 aa, Artificial Sequence
  Fusion protein_N-Fc
RSKQRRPQGLPNNTASWFTALTQHGKEDLKFPRGQGVPINTNSSPDDQIGYYRRATRRIRGGDGKMKDLSPRWYFYYLGTGPEAGLPYGANKDGIIWVATEGALNTPKDHIGTRNPANNAAIVLQLPQGTTLPKGFYAEGSRGGSQASSRSSSRSRGGGGSGGGGSGGGGSEPKSSDKTHTCPPCPAPELLGGPSVFLFPPKPKDTLMISRTPEVTCVVVDVSHEDPEVKFNWYVDGVEVHNAKTKPREEQYNSTYRVVSVLTVLHQDWLNGKEYKCKVSNKALPAPIEKTISKAKGQPREPQVYTLPPSRDELTKNQVSLTCLVKGFYPSDIAVEWESNGQPENNYKTTPPVLDSDGSFFLYSKLTVDKSRWQQGNVFSCSVMHEALHNHYTQKSLSLSPG

SEQ ID NO: 43 - protein, 465 aa, Artificial Sequence
  Fusion protein_RBDm(Q175A, N183A)-Fc
RVQPTESIVRFPNITNLCPFGEVFNATRFASVYAWNRKRISNCVADYSVLYNSASFSTFKCYGVSPTKLNDLCFTNVYADSFVIRGDEVRQIAPGQTGKIADYNYKLPDDFTGCVIAWNSNNLDSKVGGNYNYLYRLFRKSNLKPFERDISTEIYQAGSTPCNGVEGFNCYFPLASYGFQPTAGVGYQPYRVVVLSFELLHAPATVCGPKKSTNLVKNKGGGGSGGGGSGGGGSEPKSSDKTHTCPPCPAPELLGGPSVFLFPPKPKDTLMISRTPEVTCVVVDVSHEDPEVKFNWYVDGVEVHNAKTKPREEQYNSTYRVVSVLTVLHQDWLNGKEYKCKVSNKALPAPIEKTISKAKGQPREPQVYTLPPSRDELTKNQVSLTCLVKGFYPSDIAVEWESNGQPENNYKTTPPVLDSDGSFFLYSKLTVDKSRWQQGNVFSCSVMHEALHNHYTQKSLSLSPG

SEQ ID NO: 44 - protein, 465 aa, Artificial Sequence
  Fusion protein_RBDm(G164A, V165A, Q175A, S176A, N183A)-Fc
RVQPTESIVRFPNITNLCPFGEVFNATRFASVYAWNRKRISNCVADYSVLYNSASFSTFKCYGVSPTKLNDLCFTNVYADSFVIRGDEVRQIAPGQTGKIADYNYKLPDDFTGCVIAWNSNNLDSKVGGNYNYLYRLFRKSNLKPFERDISTEIYQAGSTPCNAAEGFNCYFPLAAYGFQPTAGVGYQPYRVVVLSFELLHAPATVCGPKKSTNLVKNKGGGGSGGGGSGGGGSEPKSSDKTHTCPPCPAPELLGGPSVFLFPPKPKDTLMISRTPEVTCVVVDVSHEDPEVKFNWYVDGVEVHNAKTKPREEQYNSTYRVVSVLTVLHQDWLNGKEYKCKVSNKALPAPIEKTISKAKGQPREPQVYTLPPSRDELTKNQVSLTCLVKGFYPSDIAVEWESNGQPENNYKTTPPVLDSDGSFFLYSKLTVDKSRWQQGNVFSCSVMHEALHNHYTQKSLSLSPG

SEQ ID NO: 45 - protein, 485 aa, Artificial Sequence
  Fusion protein_Fc-RBDm(L137A, F168A)
GGGGSGGGGSGGGGSEPKSSDKTHTCPPCPAPELLGGPSVFLFPPKPKDTLMISRTPEVTCVVVDVSHEDPEVKFNWYVDGVEVHNAKTKPREEQYNSTYRVVSVLTVLHQDWLNGKEYKCKVSNKALPAPIEKTISKAKGQPREPQVYTLPPSRDELTKNQVSLTCLVKGFYPSDIAVEWESNGQPENNYKTTPPVLDSDGSFFLYSKLTVDKSRWQQGNVFSCSVMHEALHNHYTQKSLSLSPGGGGGSGGGGSGGGGSGGGGSRVQPTESIVRFPNITNLCPFGEVFNATRFASVYAWNRKRISNCVADYSVLYNSASFSTFKCYGVSPTKLNDLCFTNVYADSFVIRGDEVRQIAPGQTGKIADYNYKLPDDFTGCVIAWNSNNLDSKVGGNYNYLYRAFRKSNLKPFERDISTEIYQAGSTPCNGVEGANCYFPLQSYGFQPTNGVGYQPYRVVVLSFELLHAPATVCGPKKSTNLVKNK

SEQ ID NO: 46 - protein, 485 aa, Artificial Sequence
  Fusion protein_Fc-RBDm(L137A, G164A, V165A, F168A, Q175A, S176A, N183A)
GGGGSGGGGSGGGGSEPKSSDKTHTCPPCPAPELLGGPSVFLFPPKPKDTLMISRTPEVTCVVVDVSHEDPEVKFNWYVDGVEVHNAKTKPREEQYNSTYRVVSVLTVLHQDWLNGKEYKCKVSNKALPAPIEKTISKAKGQPREPQVYTLPPSRDELTKNQVSLTCLVKGFYPSDIAVEWESNGQPENNYKTTPPVLDSDGSFFLYSKLTVDKSRWQQGNVFSCSVMHEALHNHYTQKSLSLSPGGGGGSGGGGSGGGGSGGGGSRVQPTESIVRFPNITNLCPFGEVFNATRFASVYAWNRKRISNCVADYSVLYNSASFSTFKCYGVSPTKLNDLCFTNVYADSFVIRGDEVRQIAPGQTGKIADYNYKLPDDFTGCVIAWNSNNLDSKVGGNYNYLYRAFRKSNLKPFERDISTEIYQAGSTPCNAAEGANCYFPLAAYGFQPTAGVGYQPYRVVVLSFELLHAPATVCGPKKSTNLVKNK

SEQ ID NO: 47 - protein, 465 aa, Artificial Sequence
  Fusion protein_RBDm(L137A, F168A)-Fc
RVQPTESIVRFPNITNLCPFGEVFNATRFASVYAWNRKRISNCVADYSVLYNSASFSTFKCYGVSPTKLNDLCFTNVYADSFVIRGDEVRQIAPGQTGKIADYNYKLPDDFTGCVIAWNSNNLDSKVGGNYNYLYRAFRKSNLKPFERDISTEIYQAGSTPCNGVEGANCYFPLQSYGFQPTNGVGYQPYRVVVLSFELLHAPATVCGPKKSTNLVKNKGGGGSGGGGSGGGGSEPKSSDKTHTCPPCPAPELLGGPSVFLFPPKPKDTLMISRTPEVTCVVVDVSHEDPEVKFNWYVDGVEVHNAKTKPREEQYNSTYRVVSVLTVLHQDWLNGKEYKCKVSNKALPAPIEKTISKAKGQPREPQVYTLPPSRDELTKNQVSLTCLVKGFYPSDIAVEWESNGQPENNYKTTPPVLDSDGSFFLYSKLTVDKSRWQQGNVFSCSVMHEALHNHYTQKSLSLSPG

SEQ ID NO: 48 - protein, 465 aa, Artificial Sequence
  Fusion protein_RBDm(L137A, G164A, V165A, F168A, Q175A, S176A, N183A)-Fc
RVQPTESIVRFPNITNLCPFGEVFNATRFASVYAWNRKRISNCVADYSVLYNSASFSTFKCYGVSPTKLNDLCFTNVYADSFVIRGDEVRQIAPGQTGKIADYNYKLPDDFTGCVIAWNSNNLDSKVGGNYNYLYRAFRKSNLKPFERDISTEIYQAGSTPCNAAEGANCYFPLAAYGFQPTAGVGYQPYRVVVLSFELLHAPATVCGPKKSTNLVKNKGGGGSGGGGSGGGGSEPKSSDKTHTCPPCPAPELLGGPSVFLFPPKPKDTLMISRTPEVTCVVVDVSHEDPEVKFNWYVDGVEVHNAKTKPREEQYNSTYRVVSVLTVLHQDWLNGKEYKCKVSNKALPAPIEKTISKAKGQPREPQVYTLPPSRDELTKNQVSLTCLVKGFYPSDIAVEWESNGQPENNYKTTPPVLDSDGSFFLYSKLTVDKSRWQQGNVFSCSVMHEALHNHYTQKSLSLSPG

SEQ ID NO: 49 - protein, 641 aa, Artificial Sequence
  Fusion protein_GIC-1114
RSKQRRPQGLPNNTASWFTALTQHGKEDLKFPRGQGVPINTNSSPDDQIGYYRRATRRIRGGDGKMKDLSPRWYFYYLGTGPEAGLPYGANKDGIIWVATEGALNTPKDHIGTRNPANNAAIVLQLPQGTTLPKGFYAEGSRGGSQASSRSSSRSRGGGGSGGGGSGGGGSEPKSSDKTHTCPPCPAPELLGGPSVFLFPPKPKDTLMISRTPEVTCVVVDVSHEDPEVKFNWYVDGVEVHNAKTKPREEQYNSTYRVVSVLTVLHQDWLNGKEYKCKVSNKALPAPIEKTISKAKGQPREPQVYTLPPSRDELTKNQVSLTCLVKGFYPSDIAVEWESNGQPENNYKTTPPVLDSDGSFFLYSKLTVDKSRWQQGNVFSCSVMHEALHNHYTQKSLSLSPGGGGGSGGGGSGGGGSGGGGSRVQPTESIVRFPNITNLCPFGEVFNATRFASVYAWNRKRISNCVADYSVLYNSASFSTFKCYGVSPTKLNDLCFTNVYADSFVIRGDEVRQIAPGQTGKIADYNYKLPDDFTGCVIAWNSNNLDSKVGGNYNYLYRLFRKSNLKPFERDISTEIYQAGSTPCNGVEGFNCYFPLQSYGFQPTNGVGYQPYRVVVLSFELLHAPATVCGPKKSTNLVKNK

SEQ ID NO: 50 - protein, 641 aa, Artificial Sequence
  Fusion protein_GIC-1114m(L137A, F168A)
RSKQRRPQGLPNNTASWFTALTQHGKEDLKFPRGQGVPINTNSSPDDQIGYYRRATRRIRGGDGKMKDLSPRWYFYYLGTGPEAGLPYGANKDGIIWVATEGALNTPKDHIGTRNPANNAAIVLQLPQGTTLPKGFYAEGSRGGSQASSRSSSRSRGGGGSGGGGSGGGGSEPKSSDKTHTCPPCPAPELLGGPSVFLFPPKPKDTLMISRTPEVTCVVVDVSHEDPEVKFNWYVDGVEVHNAKTKPREEQYNSTYRVVSVLTVLHQDWLNGKEYKCKVSNKALPAPIEKTISKAKGQPREPQVYTLPPSRDELTKNQVSLTCLVKGFYPSDIAVEWESNGQPENNYKTTPPVLDSDGSFFLYSKLTVDKSRWQQGNVFSCSVMHEALHNHYTQKSLSLSPGGGGGSGGGGSGGGGSGGGGSRVQPTESIVRFPNITNLCPFGEVFNATRFASVYAWNRKRISNCVADYSVLYNSASFSTFKCYGVSPTKLNDLCFTNVYADSFVIRGDEVRQIAPGQTGKIADYNYKLPDDFTGCVIAWNSNNLDSKVGGNYNYLYRAFRKSNLKPFERDISTEIYQAGSTPCNGVEGANCYFPLQSYGFQPTNGVGYQPYRVVVLSFELLHAPATVCGPKKSTNLVKNK

SEQ ID NO: 51 - protein, 641 aa, Artificial Sequence
  Fusion protein_GIC-1114m(L137A)
RSKQRRPQGLPNNTASWFTALTQHGKEDLKFPRGQGVPINTNSSPDDQIGYYRRATRRIRGGDGKMKDLSPRWYFYYLGTGPEAGLPYGANKDGIIWVATEGALNTPKDHIGTRNPANNAAIVLQLPQGTTLPKGFYAEGSRGGSQASSRSSSRSRGGGGSGGGGSGGGGSEPKSSDKTHTCPPCPAPELLGGPSVFLFPPKPKDTLMISRTPEVTCVVVDVSHEDPEVKFNWYVDGVEVHNAKTKPREEQYNSTYRVVSVLTVLHQDWLNGKEYKCKVSNKALPAPIEKTISKAKGQPREPQVYTLPPSRDELTKNQVSLTCLVKGFYPSDIAVEWESNGQPENNYKTTPPVLDSDGSFFLYSKLTVDKSRWQQGNVFSCSVMHEALHNHYTQKSLSLSPGGGGGSGGGGSGGGGSGGGGSRVQPTESIVRFPNITNLCPFGEVFNATRFASVYAWNRKRISNCVADYSVLYNSASFSTFKCYGVSPTKLNDLCFTNVYADSFVIRGDEVRQIAPGQTGKIADYNYKLPDDFTGCVIAWNSNNLDSKVGGNYNYLYRAFRKSNLKPFERDISTEIYQAGSTPCNGVEGFNCYFPLQSYGFQPTNGVGYQPYRVVVLSFELLHAPATVCGPKKSTNLVKNK

SEQ ID NO: 52 - protein, 641 aa, Artificial Sequence
  Fusion protein_GIC-1114m(F168A)
RSKQRRPQGLPNNTASWFTALTQHGKEDLKFPRGQGVPINTNSSPDDQIGYYRRATRRIRGGDGKMKDLSPRWYFYYLGTGPEAGLPYGANKDGIIWVATEGALNTPKDHIGTRNPANNAAIVLQLPQGTTLPKGFYAEGSRGGSQASSRSSSRSRGGGGSGGGGSGGGGSEPKSSDKTHTCPPCPAPELLGGPSVFLFPPKPKDTLMISRTPEVTCVVVDVSHEDPEVKFNWYVDGVEVHNAKTKPREEQYNSTYRVVSVLTVLHQDWLNGKEYKCKVSNKALPAPIEKTISKAKGQPREPQVYTLPPSRDELTKNQVSLTCLVKGFYPSDIAVEWESNGQPENNYKTTPPVLDSDGSFFLYSKLTVDKSRWQQGNVFSCSVMHEALHNHYTQKSLSLSPGGGGGSGGGGSGGGGSGGGGSRVQPTESIVRFPNITNLCPFGEVFNATRFASVYAWNRKRISNCVADYSVLYNSASFSTFKCYGVSPTKLNDLCFTNVYADSFVIRGDEVRQIAPGQTGKIADYNYKLPDDFTGCVIAWNSNNLDSKVGGNYNYLYRLFRKSNLKPFERDISTEIYQAGSTPCNGVEGANCYFPLQSYGFQPTNGVGYQPYRVVVLSFELLHAPATVCGPKKSTNLVKNK

SEQ ID NO: 53 - protein, 641 aa, Artificial Sequence
  Fusion protein_GIC-1114m(G184D)
RSKQRRPQGLPNNTASWFTALTQHGKEDLKFPRGQGVPINTNSSPDDQIGYYRRATRRIRGGDGKMKDLSPRWYFYYLGTGPEAGLPYGANKDGIIWVATEGALNTPKDHIGTRNPANNAAIVLQLPQGTTLPKGFYAEGSRGGSQASSRSSSRSRGGGGSGGGGSGGGGSEPKSSDKTHTCPPCPAPELLGGPSVFLFPPKPKDTLMISRTPEVTCVVVDVSHEDPEVKFNWYVDGVEVHNAKTKPREEQYNSTYRVVSVLTVLHQDWLNGKEYKCKVSNKALPAPIEKTISKAKGQPREPQVYTLPPSRDELTKNQVSLTCLVKGFYPSDIAVEWESNGQPENNYKTTPPVLDSDGSFFLYSKLTVDKSRWQQGNVFSCSVMHEALHNHYTQKSLSLSPGGGGGSGGGGSGGGGSGGGGSRVQPTESIVRFPNITNLCPFGEVFNATRFASVYAWNRKRISNCVADYSVLYNSASFSTFKCYGVSPTKLNDLCFTNVYADSFVIRGDEVRQIAPGQTGKIADYNYKLPDDFTGCVIAWNSNNLDSKVGGNYNYLYRLFRKSNLKPFERDISTEIYQAGSTPCNGVEGFNCYFPLQSYGFQPTNDVGYQPYRVVVLSFELLHAPATVCGPKKSTNLVKNK

SEQ ID NO: 54 - protein, 641 aa, Artificial Sequence
  Fusion protein_GIC-1114m(L137A, G164A, V165A, F168A, Q175A, S176A, N183A)
RSKQRRPQGLPNNTASWFTALTQHGKEDLKFPRGQGVPINTNSSPDDQIGYYRRATRRIRGGDGKMKDLSPRWYFYYLGTGPEAGLPYGANKDGIIWVATEGALNTPKDHIGTRNPANNAAIVLQLPQGTTLPKGFYAEGSRGGSQASSRSSSRSRGGGGSGGGGSGGGGSEPKSSDKTHTCPPCPAPELLGGPSVFLFPPKPKDTLMISRTPEVTCVVVDVSHEDPEVKFNWYVDGVEVHNAKTKPREEQYNSTYRVVSVLTVLHQDWLNGKEYKCKVSNKALPAPIEKTISKAKGQPREPQVYTLPPSRDELTKNQVSLTCLVKGFYPSDIAVEWESNGQPENNYKTTPPVLDSDGSFFLYSKLTVDKSRWQQGNVFSCSVMHEALHNHYTQKSLSLSPGGGGGSGGGGSGGGGSGGGGSRVQPTESIVRFPNITNLCPFGEVFNATRFASVYAWNRKRISNCVADYSVLYNSASFSTFKCYGVSPTKLNDLCFTNVYADSFVIRGDEVRQIAPGQTGKIADYNYKLPDDFTGCVIAWNSNNLDSKVGGNYNYLYRAFRKSNLKPFERDISTEIYQAGSTPCNAAEGANCYFPLAAYGFQPTAGVGYQPYRVVVLSFELLHAPATVCGPKKSTNLVKNK

SEQ ID NO: 55 - protein, 641 aa, Artificial Sequence
  Fusion protein_GIC-1114N
RVQPTESIVRFPNITNLCPFGEVFNATRFASVYAWNRKRISNCVADYSVLYNSASFSTFKCYGVSPTKLNDLCFTNVYADSFVIRGDEVRQIAPGQTGKIADYNYKLPDDFTGCVIAWNSNNLDSKVGGNYNYLYRLFRKSNLKPFERDISTEIYQAGSTPCNGVEGFNCYFPLQSYGFQPTNGVGYQPYRVVVLSFELLHAPATVCGPKKSTNLVKNKGGGGSGGGGSGGGGSEPKSSDKTHTCPPCPAPELLGGPSVFLFPPKPKDTLMISRTPEVTCVVVDVSHEDPEVKFNWYVDGVEVHNAKTKPREEQYNSTYRVVSVLTVLHQDWLNGKEYKCKVSNKALPAPIEKTISKAKGQPREPQVYTLPPSRDELTKNQVSLTCLVKGFYPSDIAVEWESNGQPENNYKTTPPVLDSDGSFFLYSKLTVDKSRWQQGNVFSCSVMHEALHNHYTQKSLSLSPGGGGGSGGGGSGGGGSGGGGSRSKQRRPQGLPNNTASWFTALTQHGKEDLKFPRGQGVPINTNSSPDDQIGYYRRATRRIRGGDGKMKDLSPRWYFYYLGTGPEAGLPYGANKDGIIWVATEGALNTPKDHIGTRNPANNAAIVLQLPQGTTLPKGFYAEGSRGGSQASSRSSSRSR

SEQ ID NO: 56 - protein, 641 aa, Artificial Sequence
  Fusion protein_GIC-1114Nm(L137A, F168A)
RVQPTESIVRFPNITNLCPFGEVFNATRFASVYAWNRKRISNCVADYSVLYNSASFSTFKCYGVSPTKLNDLCFTNVYADSFVIRGDEVRQIAPGQTGKIADYNYKLPDDFTGCVIAWNSNNLDSKVGGNYNYLYRAFRKSNLKPFERDISTEIYQAGSTPCNGVEGANCYFPLQSYGFQPTNGVGYQPYRVVVLSFELLHAPATVCGPKKSTNLVKNKGGGGSGGGGSGGGGSEPKSSDKTHTCPPCPAPELLGGPSVFLFPPKPKDTLMISRTPEVTCVVVDVSHEDPEVKFNWYVDGVEVHNAKTKPREEQYNSTYRVVSVLTVLHQDWLNGKEYKCKVSNKALPAPIEKTISKAKGQPREPQVYTLPPSRDELTKNQVSLTCLVKGFYPSDIAVEWESNGQPENNYKTTPPVLDSDGSFFLYSKLTVDKSRWQQGNVFSCSVMHEALHNHYTQKSLSLSPGGGGGSGGGGSGGGGSGGGGSRSKQRRPQGLPNNTASWFTALTQHGKEDLKFPRGQGVPINTNSSPDDQIGYYRRATRRIRGGDGKMKDLSPRWYFYYLGTGPEAGLPYGANKDGIIWVATEGALNTPKDHIGTRNPANNAAIVLQLPQGTTLPKGFYAEGSRGGSQASSRSSSRSR

SEQ ID NO: 57 - protein, 773 aa, Artificial Sequence
  Fusion protein_GIC-1132m(L137A, F168A)
RLFARTRSMWSFNPETNILLNVPLHGTILTRPLLESELVIGAVILRGHLRIAGHHLGRCDIKDLPKEITVATSRTLSYYKLGASQRVAGDSGFAAYSRYRIGNYKLNTDHSSSSDNIALLVQGGGGSGGGGSRSKQRRPQGLPNNTASWFTALTQHGKEDLKFPRGQGVPINTNSSPDDQIGYYRRATRRIRGGDGKMKDLSPRWYFYYLGTGPEAGLPYGANKDGIIWVATEGALNTPKDHIGTRNPANNAAIVLQLPQGTTLPKGFYAEGSRGGSQASSRSSSRSRGGGGSGGGGSGGGGSEPKSSDKTHTCPPCPAPELLGGPSVFLFPPKPKDTLMISRTPEVTCVVVDVSHEDPEVKFNWYVDGVEVHNAKTKPREEQYNSTYRVVSVLTVLHQDWLNGKEYKCKVSNKALPAPIEKTISKAKGQPREPQVYTLPPSRDELTKNQVSLTCLVKGFYPSDIAVEWESNGQPENNYKTTPPVLDSDGSFFLYSKLTVDKSRWQQGNVFSCSVMHEALHNHYTQKSLSLSPGGGGGSGGGGSGGGGSGGGGSRVQPTESIVRFPNITNLCPFGEVFNATRFASVYAWNRKRISNCVADYSVLYNSASFSTFKCYGVSPTKLNDLCFTNVYADSFVIRGDEVRQIAPGQTGKIADYNYKLPDDFTGCVIAWNSNNLDSKVGGNYNYLYRAFRKSNLKPFERDISTEIYQAGSTPCNGVEGANCYFPLQSYGFQPTNGVGYQPYRVVVLSFELLHAPATVCGPKKSTNLVKNK

SEQ ID NO: 58 - protein, 773 aa, Artificial Sequence
  Fusion protein_GIC-1114Nm(L137A, F168A)
RSKQRRPQGLPNNTASWFTALTQHGKEDLKFPRGQGVPINTNSSPDDQIGYYRRATRRIRGGDGKMKDLSPRWYFYYLGTGPEAGLPYGANKDGIIWVATEGALNTPKDHIGTRNPANNAAIVLQLPQGTTLPKGFYAEGSRGGSQASSRSSSRSRGGGGSGGGGSRLFARTRSMWSFNPETNILLNVPLHGTILTRPLLESELVIGAVILRGHLRIAGHHLGRCDIKDLPKEITVATSRTLSYYKLGASQRVAGDSGFAAYSRYRIGNYKLNTDHSSSSDNIALLVQGGGGSGGGGSGGGGSEPKSSDKTHTCPPCPAPELLGGPSVFLFPPKPKDTLMISRTPEVTCVVVDVSHEDPEVKFNWYVDGVEVHNAKTKPREEQYNSTYRVVSVLTVLHQDWLNGKEYKCKVSNKALPAPIEKTISKAKGQPREPQVYTLPPSRDELTKNQVSLTCLVKGFYPSDIAVEWESNGQPENNYKTTPPVLDSDGSFFLYSKLTVDKSRWQQGNVFSCSVMHEALHNHYTQKSLSLSPGGGGGSGGGGSGGGGSGGGGSRVQPTESIVRFPNITNLCPFGEVFNATRFASVYAWNRKRISNCVADYSVLYNSASFSTFKCYGVSPTKLNDLCFTNVYADSFVIRGDEVRQIAPGQTGKIADYNYKLPDDFTGCVIAWNSNNLDSKVGGNYNYLYRAFRKSNLKPFERDISTEIYQAGSTPCNGVEGANCYFPLQSYGFQPTNGVGYQPYRVVVLSFELLHAPATVCGPKKSTNLVKNK

SEQ ID NO: 59 - protein, 780 aa, Artificial Sequence
  Fusion protein_GIC-1151
RVQPTESIVRFPNITNLCPFGEVFNATRFASVYAWNRKRISNCVADYSVLYNSASFSTFKCYGVSPTKLNDLCFTNVYADSFVIRGDEVRQIAPGQTGKIADYNYKLPDDFTGCVIAWNSNNLDSKVGGNYNYLYRLFRKSNLKPFERDISTEIYQAGSTPCNGVEGFNCYFPLQSYGFQPTNGVGYQPYRVVVLSFELLHAPATVCGPKKSTNLVKNKGGSGGSGGSRSKQRRPQGLPNNTASWFTALTQHGKEDLKFPRGQGVPINTNSSPDDQIGYYRRATRRIRGGDGKMKDLSPRWYFYYLGTGPEAGLPYGANKDGIIWVATEGALNTPKDHIGTRNPANNAAIVLQLPQGTTLPKGFYAEGSRGGSQASSRSSSRSRGGSGGSGGSGGSRSKQRRPQGLPNNTASWFTALTQHGKEDLKFPRGQGVPINTNSSPDDQIGYYRRATRRIRGGDGKMKDLSPRWYFYYLGTGPEAGLPYGANKDGIIWVATEGALNTPKDHIGTRNPANNAAIVLQLPQGTTLPKGFYAEGSRGGSQASSRSSSRSRGGSGGSGGSRVQPTESIVRFPNITNLCPFGEVFNATRFASVYAWNRKRISNCVADYSVLYNSASFSTFKCYGVSPTKLNDLCFTNVYADSFVIRGDEVRQIAPGQTGKIADYNYKLPDDFTGCVIAWNSNNLDSKVGGNYNYLYRLFRKSNLKPFERDISTEIYQAGSTPCNGVEGFNCYFPLQSYGFQPTNGVGYQPYRVVVLSFELLHAPATVCGPKKSTNLVKNK

SEQ ID NO: 60 - protein, 780 aa, Artificial Sequence
  Fusion protein_GIC-1151m(L137A, F168A)
RVQPTESIVRFPNITNLCPFGEVFNATRFASVYAWNRKRISNCVADYSVLYNSASFSTFKCYGVSPTKLNDLCFTNVYADSFVIRGDEVRQIAPGQTGKIADYNYKLPDDFTGCVIAWNSNNLDSKVGGNYNYLYRAFRKSNLKPFERDISTEIYQAGSTPCNGVEGANCYFPLQSYGFQPTNGVGYQPYRVVVLSFELLHAPATVCGPKKSTNLVKNKGGSGGSGGSRSKQRRPQGLPNNTASWFTALTQHGKEDLKFPRGQGVPINTNSSPDDQIGYYRRATRRIRGGDGKMKDLSPRWYFYYLGTGPEAGLPYGANKDGIIWVATEGALNTPKDHIGTRNPANNAAIVLQLPQGTTLPKGFYAEGSRGGSQASSRSSSRSRGGSGGSGGSGGSRSKQRRPQGLPNNTASWFTALTQHGKEDLKFPRGQGVPINTNSSPDDQIGYYRRATRRIRGGDGKMKDLSPRWYFYYLGTGPEAGLPYGANKDGIIWVATEGALNTPKDHIGTRNPANNAAIVLQLPQGTTLPKGFYAEGSRGGSQASSRSSSRSRGGSGGSGGSRVQPTESIVRFPNITNLCPFGEVFNATRFASVYAWNRKRISNCVADYSVLYNSASFSTFKCYGVSPTKLNDLCFTNVYADSFVIRGDEVRQIAPGQTGKIADYNYKLPDDFTGCVIAWNSNNLDSKVGGNYNYLYRAFRKSNLKPFERDISTEIYQAGSTPCNGVEGANCYFPLQSYGFQPTNGVGYQPYRVVVLSFELLHAPATVCGPKKSTNLVKNK

SEQ ID NO: 61 - DNA, 738 bp, Artificial Sequence
  Fusion protein_DNA sequence_IgG1 Fc
ggcggcggaggatccggcggtggtggttccggcggaggcggttctgaacctaagtcctccgacaagacccacacctgtcctccatgtcctgctccagaactgctcggcggaccttccgtgtttctgttcccacctaagccaaaggacaccctgatgatcagcagaacccctgaagtgacctgcgtggtggtggatgtgtctcacgaggaccccgaagtgaagttcaattggtacgtggacggcgtggaagtgcacaacgccaagaccaagcctagagaggaacagtacaactccacctacagagtggtgtccgtgctgaccgtgctgcaccaggattggctgaacggcaaagagtacaagtgcaaggtgtccaacaaggccctgcctgctcctatcgaaaagaccatctccaaggccaagggccagcctagggaaccccaggtttacacactgcctccatctcgggacgagctgaccaagaatcaggtgtccctgacctgtctggtcaagggcttctacccttccgatatcgccgtggaatgggagagcaatggccagcctgagaacaactacaagacaacccctcctgtgctggactccgacggctcattcttcctgtatagcaagctgacagtggacaagtcccggtggcagcagggcaacgtgttctcctgttctgtgatgcacgaggccctgcacaaccactacacccagaagagtctgtccttgagcccgggc

SEQ ID NO: 62 - DNA, 1395 bp, Artificial Sequence
  Fusion protein_DNA sequence_RBDwt-Fc
agagttcagcctaccgagtccatcgtgcggttccccaacatcaccaacctgtgtcctttcggcgaggtgttcaacgctaccagattcgcctctgtgtacgcctggaaccggaagcggatctctaactgcgtggccgactactccgtgctgtacaactctgcctccttcagcaccttcaagtgctacggcgtgtcccctaccaagctgaacgacctgtgcttcaccaacgtgtacgccgactccttcgtgatcaggggcgacgaagttcggcagatcgctcctggacagaccggcaagatcgccgactacaattacaagctgcccgacgacttcaccggctgcgtgatcgcttggaactccaacaacctggactccaaagtcggcggcaactacaactacctgtaccggctgttccggaagtccaacctgaagcctttcgagcgggacatctccaccgagatctaccaggctggcagcaccccttgcaatggcgtcgagggcttcaactgctacttcccactgcagtcctacggcttccagcctaccaatggcgtgggctaccagccttatagagtggtggtgctgtccttcgagctgctgcatgctcctgctaccgtgtgcggccctaagaaatctaccaacctggtcaagaacaagggcggcggaggatccggcggtggtggttccggcggaggcggttctgaacctaagtcctccgacaagacccacacctgtcctccatgtcctgctccagaactgctcggcggaccttccgtgtttctgttcccacctaagccaaaggacaccctgatgatcagcagaacccctgaagtgacctgcgtggtggtggatgtgtctcacgaggaccccgaagtgaagttcaattggtacgtggacggcgtggaagtgcacaacgccaagaccaagcctagagaggaacagtacaactccacctacagagtggtgtccgtgctgaccgtgctgcaccaggattggctgaacggcaaagagtacaagtgcaaggtgtccaacaaggccctgcctgctcctatcgaaaagaccatctccaaggccaagggccagcctagggaaccccaggtttacacactgcctccatctcgggacgagctgaccaagaatcaggtgtccctgacctgtctggtcaagggcttctacccttccgatatcgccgtggaatgggagagcaatggccagcctgagaacaactacaagacaacccctcctgtgctggactccgacggctcattcttcctgtatagcaagctgacagtggacaagtcccggtggcagcagggcaacgtgttctcctgttctgtgatgcacgaggccctgcacaaccactacacccagaagagtctgtccttgagcccgggc

SEQ ID NO: 63 - DNA, 1455 bp, Artificial Sequence
  Fusion protein_DNA sequence_Fc-RBDwt
ggcggcggaggatccggcggtggtggttccggcggaggcggttctgaacctaagtcctccgacaagacccacacctgtcctccatgtcctgctccagaactgctcggcggaccttccgtgtttctgttcccacctaagccaaaggacaccctgatgatcagcagaacccctgaagtgacctgcgtggtggtggatgtgtctcacgaggaccccgaagtgaagttcaattggtacgtggacggcgtggaagtgcacaacgccaagaccaagcctagagaggaacagtacaactccacctacagagtggtgtccgtgctgaccgtgctgcaccaggattggctgaacggcaaagagtacaagtgcaaggtgtccaacaaggccctgcctgctcctatcgaaaagaccatctccaaggccaagggccagcctagggaaccccaggtttacacactgcctccatctcgggacgagctgaccaagaatcaggtgtccctgacctgtctggtcaagggcttctacccttccgatatcgccgtggaatgggagagcaatggccagcctgagaacaactacaagacaacccctcctgtgctggactccgacggctcattcttcctgtatagcaagctgacagtggacaagtcccggtggcagcagggcaacgtgttctcctgttctgtgatgcacgaggccctgcacaaccactacacccagaagagtctgtccttgagcccgggcggtggcggcggttcaggcggcggtggaagtggcggtggcggatctggcggaggtggtagtagagttcagcctaccgagtccatcgtgcggttccccaacatcaccaacctgtgtcctttcggcgaggtgttcaacgctaccagattcgcctctgtgtacgcctggaaccggaagcggatctctaactgcgtggccgactactccgtgctgtacaactctgcctccttcagcaccttcaagtgctacggcgtgtcccctaccaagctgaacgacctgtgcttcaccaacgtgtacgccgactccttcgtgatcaggggcgacgaagttcggcagatcgctcctggacagaccggcaagatcgccgactacaattacaagctgcccgacgacttcaccggctgcgtgatcgcttggaactccaacaacctggactccaaagtcggcggcaactacaactacctgtaccggctgttccggaagtccaacctgaagcctttcgagcgggacatctccaccgagatctaccaggctggcagcaccccttgcaatggcgtcgagggcttcaactgctacttcccactgcagtcctacggcttccagcctaccaatggcgtgggctaccagccttatagagtggtggtgctgtccttcgagctgctgcatgctcctgctaccgtgtgcggccctaagaaatctaccaacctggtcaagaacaag

SEQ ID NO: 64 - DNA, 1206 bp, Artificial Sequence
  Fusion protein_DNA sequence_N-Fc
cggtctaagcagagaaggcctcagggcctgcctaacaataccgcctcctggtttaccgctctgacccagcacggcaaagaggacctgaagttccctagaggacagggcgtgcccatcaacaccaactctagccctgacgaccagatcggctactacagacgggccaccagaagaatcagaggcggcgacggcaagatgaaggacctgtctcctcggtggtacttctactacctcggcaccggaccagaggctggattgccttatggcgccaacaaggacggcatcatctgggttgcaacagagggcgctctgaacacccctaaggaccacatcggcacccggaatcctgccaacaatgctgccattgtgctgcagctgccacagggcacaacactgcctaagggcttttacgccgagggctctagaggcggctctcaggcctcttccagatcctccagtagatcacgtggcggcggaggatccggtggtggtggatctggtggcggaggctctgaacctaagtcctccgacaagacccacacctgtcctccatgtcctgctccagaactgctcggcggaccttccgtgtttctgttcccacctaagccaaaggacaccctgatgatcagcagaacccctgaagtgacctgcgtggtggtggatgtgtctcacgaggaccccgaagtgaagttcaattggtacgtggacggcgtggaagtgcacaacgccaagaccaagcctagagaggaacagtacaactccacctacagagtggtgtccgtgctgaccgtgctgcaccaggattggctgaacggcaaagagtacaagtgcaaggtgtccaacaaggccctgcctgctcctatcgaaaagaccatctccaaggccaagggccagcctagggaaccccaggtttacacactgcctccatctcgggacgagctgaccaagaatcaggtgtccctgacctgtctggtcaagggcttctacccttccgatatcgccgtggaatgggagagcaatggccagcctgagaacaactacaagacaacccctcctgtgctggactccgacggctcattcttcctgtatagcaagctgacagtggacaagtcccggtggcagcagggcaacgtgttctcctgttctgtgatgcacgaggccctgcacaaccactacacccagaagagtctgtccttgagcccgggc

SEQ ID NO: 65 - DNA, 1395 bp, Artificial Sequence
  Fusion protein_DNA sequence_RBDm(Q175A, N183A)-Fc
agagtgcagcctaccgagtctatcgtgcggttccccaacatcaccaacctgtgtcctttcggcgaggtgttcaacgccaccagattcgcctctgtgtacgcctggaaccggaagcggatctctaactgcgtggccgactactccgtgctgtacaactccgcctccttcagcaccttcaagtgctacggcgtgtcccctaccaagctgaacgacctgtgcttcaccaacgtgtacgccgactccttcgtgatcagaggcgacgaagtgcggcagatcgctcctggacagaccggcaagatcgccgactacaactacaagctgcccgacgacttcaccggctgtgtgatcgcttggaactccaacaacctggactccaaagtcggcggcaactacaattacctgtaccggctgttccggaagtccaacctgaagcctttcgagcgggacatctccaccgagatctaccaggctggcagcaccccttgtaatggcgtggaaggcttcaactgctacttccctctggcctcctacggcttccaacctacagctggcgtgggctaccagccttacagagtggtggtgctgtccttcgagctgctgcatgctcctgctaccgtgtgcggccctaagaaatctaccaacctggtcaagaacaagggcggcggaggatccggcggtggtggttccggcggaggcggttctgaacctaagtcctccgacaagacccacacctgtcctccatgtcctgctccagaactgctcggcggaccttccgtgtttctgttcccacctaagccaaaggacaccctgatgatcagcagaacccctgaagtgacctgcgtggtggtggatgtgtctcacgaggaccccgaagtgaagttcaattggtacgtggacggcgtggaagtgcacaacgccaagaccaagcctagagaggaacagtacaactccacctacagagtggtgtccgtgctgaccgtgctgcaccaggattggctgaacggcaaagagtacaagtgcaaggtgtccaacaaggccctgcctgctcctatcgaaaagaccatctccaaggccaagggccagcctagggaaccccaggtttacacactgcctccatctcgggacgagctgaccaagaatcaggtgtccctgacctgtctggtcaagggcttctacccttccgatatcgccgtggaatgggagagcaatggccagcctgagaacaactacaagacaacccctcctgtgctggactccgacggctcattcttcctgtatagcaagctgacagtggacaagtcccggtggcagcagggcaacgtgttctcctgttctgtgatgcacgaggccctgcacaaccactacacccagaagagtctgtccttgagcccgggc

SEQ ID NO: 66 - DNA, 1395 bp, Artificial Sequence
  Fusion protein_DNA sequence_RBDm(G164A, V165A, Q175A, S176A, N183A)-Fc
agagtgcagcctaccgagtctatcgtgcggttccccaacatcaccaacctgtgtcctttcggcgaggtgttcaacgccaccagattcgcctctgtgtacgcctggaaccggaagcggatctctaactgcgtggccgactactccgtgctgtacaactccgcctccttcagcaccttcaagtgctacggcgtgtcccctaccaagctgaacgacctgtgcttcaccaacgtgtacgccgactccttcgtgatcagaggcgacgaagtgcggcagatcgctcctggacagaccggcaagatcgccgactacaactacaagctgcccgacgacttcaccggctgtgtgatcgcttggaactccaacaacctggactccaaagtcggcggcaactacaattacctgtaccggctgttccggaagtccaacctgaagcctttcgagcgggacatctccaccgagatctaccaggctggcagcaccccttgtaatgccgccgagggcttcaactgctactttcctctggccgcctacggcttccaacctacagctggcgttggctaccagccttacagagtggtggtgctgtccttcgagctgctgcatgctcctgctaccgtgtgcggccctaagaaatctaccaacctggtcaagaacaagggcggcggaggatccggcggtggtggttccggcggaggcggttctgaacctaagtcctccgacaagacccacacctgtcctccatgtcctgctccagaactgctcggcggaccttccgtgtttctgttcccacctaagccaaaggacaccctgatgatcagcagaacccctgaagtgacctgcgtggtggtggatgtgtctcacgaggaccccgaagtgaagttcaattggtacgtggacggcgtggaagtgcacaacgccaagaccaagcctagagaggaacagtacaactccacctacagagtggtgtccgtgctgaccgtgctgcaccaggattggctgaacggcaaagagtacaagtgcaaggtgtccaacaaggccctgcctgctcctatcgaaaagaccatctccaaggccaagggccagcctagggaaccccaggtttacacactgcctccatctcgggacgagctgaccaagaatcaggtgtccctgacctgtctggtcaagggcttctacccttccgatatcgccgtggaatgggagagcaatggccagcctgagaacaactacaagacaacccctcctgtgctggactccgacggctcattcttcctgtatagcaagctgacagtggacaagtcccggtggcagcagggcaacgtgttctcctgttctgtgatgcacgaggccctgcacaaccactacacccagaagagtctgtccttgagcccgggc

SEQ ID NO: 67 - DNA, 1455 bp, Artificial Sequence
  Fusion protein_DNA sequence_Fc-RBDm(L137A, F168A)
ggcggcggaggatccggcggtggtggttccggcggaggcggttctgaacctaagtcctccgacaagacccacacctgtcctccatgtcctgctccagaactgctcggcggaccttccgtgtttctgttcccacctaagccaaaggacaccctgatgatcagcagaacccctgaagtgacctgcgtggtggtggatgtgtctcacgaggaccccgaagtgaagttcaattggtacgtggacggcgtggaagtgcacaacgccaagaccaagcctagagaggaacagtacaactccacctacagagtggtgtccgtgctgaccgtgctgcaccaggattggctgaacggcaaagagtacaagtgcaaggtgtccaacaaggccctgcctgctcctatcgaaaagaccatctccaaggccaagggccagcctagggaaccccaggtttacacactgcctccatctcgggacgagctgaccaagaatcaggtgtccctgacctgtctggtcaagggcttctacccttccgatatcgccgtggaatgggagagcaatggccagcctgagaacaactacaagacaacccctcctgtgctggactccgacggctcattcttcctgtatagcaagctgacagtggacaagtcccggtggcagcagggcaacgtgttctcctgttctgtgatgcacgaggccctgcacaaccactacacccagaagagtctgtccttgagcccgggcggtggcggcggttcaggcggcggtggaagtggcggtggcggatctggcggaggtggtagtagagtgcagcctaccgagtccatcgtgcggttccccaacatcaccaacctgtgtcctttcggcgaggtgttcaacgctaccagattcgcctctgtgtacgcctggaaccggaagcggatctctaactgcgtggccgactactccgtgctgtacaactctgcctccttcagcaccttcaagtgctacggcgtgtcccctaccaagctgaacgacctgtgcttcaccaacgtgtacgccgactccttcgtgatcaggggcgacgaagttcggcagatcgctcctggacagaccggcaagatcgccgactacaattacaagctgcccgacgacttcaccggctgcgtgatcgcttggaactccaacaacctggactccaaagtcggcggcaactacaactacctgtaccgggccttcagaaagtccaacctgaagcctttcgagcgggacatctccaccgagatctaccaggctggcagcaccccttgcaatggcgttgaaggcgccaactgctacttcccactgcagtcctacggcttccagcctaccaatggcgtgggctaccagccttatagagtggtggtgctgtccttcgagctgctgcatgctcctgctacagtgtgcggccccaagaaatctaccaacctggtcaagaacaag

SEQ ID NO: 68 - DNA, 1455 bp, Artificial Sequence
  Fusion protein_DNA sequence_Fc-RBDm(L137A, G164A, V165A, F168A, Q175A, S176A, N183A)
ggcggcggaggatccggcggtggtggttccggcggaggcggttctgaacctaagtcctccgacaagacccacacctgtcctccatgtcctgctccagaactgctcggcggaccttccgtgtttctgttccctccaaagcctaaggacaccctgatgatctctcggacccctgaagtgacctgcgtggtggtcgatgtgtctcacgaggacccagaagtgaagttcaattggtacgtggacggcgtggaagtgcacaacgccaagaccaagcctagagaggaacagtacaactccacctacagagtggtgtccgtgctgaccgtgctgcaccaggattggctgaatggcaaagagtacaagtgcaaggtgtccaacaaggccctgcctgctcctatcgaaaagaccatctccaaggccaagggccagcctagggaaccccaggtttacaccttgcctccatctcgggacgagctgaccaagaaccaggtgtccctgacctgtctggtcaagggcttctacccctccgatatcgccgtggaatgggagtctaatggccagcctgagaacaactacaagacaacccctcctgtgctggactccgacggctcattcttcctgtactccaagctgacagtggacaagtccagatggcagcagggcaacgtgttctcctgctccgtgatgcacgaggccctgcacaatcactacacacagaagtccctgtctctgtcccctggtggtggcggcggttcaggcggcggtggaagtggcggtggcggatctggcggaggtggtagtagagtgcagcctaccgagtctatcgtgcggttccccaacatcaccaacctgtgtcctttcggcgaggtgttcaacgccaccagattcgcctctgtgtacgcctggaaccggaagcggatctctaactgcgtggccgactactccgtgctgtacaactccgcctccttcagcaccttcaagtgctacggcgtgtcccctaccaagctgaacgacctgtgcttcaccaacgtgtacgccgactccttcgtgatcagaggcgacgaagtgcggcagatcgctcctggacagaccggcaagatcgccgactacaactacaagctgcccgacgacttcaccggctgtgtgatcgcttggaactccaacaacctggactccaaagtcggcggcaactacaattacctgtaccgggccttccgcaagtccaacctgaagcctttcgagcgggacatctccaccgagatctaccaggctggcagcaccccttgtaatgctgccgaaggcgccaactgctactttcctctggccgcctatggcttccagcctacagctggcgttggctaccagccttatagagtggtggtgctgtccttcgagctgctgcatgctcctgctaccgtgtgcggccctaagaaatctaccaacctggtcaagaacaaa

SEQ ID NO: 69 - DNA, 1395 bp, Artificial Sequence
  Fusion protein_DNA sequence_RBDm(L137A, F168A)-Fc
agagtgcagcctaccgagtccatcgtgcggttccccaacatcaccaacctgtgtcctttcggcgaggtgttcaacgctaccagattcgcctctgtgtacgcctggaaccggaagcggatctctaactgcgtggccgactactccgtgctgtacaactctgcctccttcagcaccttcaagtgctacggcgtgtcccctaccaagctgaacgacctgtgcttcaccaacgtgtacgccgactccttcgtgatcaggggcgacgaagttcggcagatcgctcctggacagaccggcaagatcgccgactacaattacaagctgcccgacgacttcaccggctgcgtgatcgcttggaactccaacaacctggactccaaagtcggcggcaactacaactacctgtaccgggccttcagaaagtccaacctgaagcctttcgagcgggacatctccaccgagatctaccaggctggcagcaccccttgcaatggcgttgaaggcgccaactgctacttcccactgcagtcctacggcttccagcctaccaatggcgtgggctaccagccttatagagtggtggtgctgtccttcgagctgctgcatgctcctgctacagtgtgcggccccaagaaatctaccaacctggtcaagaacaagggcggcggaggatccggcggtggtggttccggcggaggcggttctgaacctaagtcctccgacaagacccacacctgtcctccatgtcctgctccagaactgctcggcggaccttccgtgtttctgttcccacctaagccaaaggacaccctgatgatcagcagaacccctgaagtgacctgcgtggtggtggatgtgtctcacgaggaccccgaagtgaagttcaattggtacgtggacggcgtggaagtgcacaacgccaagaccaagcctagagaggaacagtacaactccacctacagagtggtgtccgtgctgaccgtgctgcaccaggattggctgaacggcaaagagtacaagtgcaaggtgtccaacaaggccctgcctgctcctatcgaaaagaccatctccaaggccaagggccagcctagggaaccccaggtttacacactgcctccatctcgggacgagctgaccaagaatcaggtgtccctgacctgtctggtcaagggcttctacccttccgatatcgccgtggaatgggagagcaatggccagcctgagaacaactacaagacaacccctcctgtgctggactccgacggctcattcttcctgtatagcaagctgacagtggacaagtcccggtggcagcagggcaacgtgttctcctgttctgtgatgcacgaggccctgcacaaccactacacccagaagagtctgtccttgagcccgggc

SEQ ID NO: 70 - DNA, 1395 bp, Artificial Sequence
  Fusion protein_DNA sequence_RBDm(L137A, G164A, V165A, F168A, Q175A, S176A, N183A)-Fc
agagtgcagcctaccgagtctatcgtgcggttccccaacatcaccaacctgtgtcctttcggcgaggtgttcaacgccaccagattcgcctctgtgtacgcctggaaccggaagcggatctctaactgcgtggccgactactccgtgctgtacaactccgcctccttcagcaccttcaagtgctacggcgtgtcccctaccaagctgaacgacctgtgcttcaccaacgtgtacgccgactccttcgtgatcagaggcgacgaagtgcggcagatcgctcctggacagaccggcaagatcgccgactacaactacaagctgcccgacgacttcaccggctgtgtgatcgcttggaactccaacaacctggactccaaagtcggcggcaactacaattacctgtaccgggccttccgcaagtccaacctgaagcctttcgagcgggacatctccaccgagatctaccaggctggcagcaccccttgtaatgctgccgaaggcgccaactgctactttcctctggccgcctatggcttccagcctacagctggcgttggctaccagccttatagagtggtggtgctgtccttcgagctgctgcatgctcctgctaccgtgtgcggccctaagaaatctaccaacctggtcaagaacaaaggcggcggaggatccggcggtggtggttccggcggaggcggttctgaacctaagtcctccgacaagacccacacctgtcctccatgtcctgctccagaactgctcggcggaccttccgtgtttctgttcccacctaagccaaaggacaccctgatgatcagcagaacccctgaagtgacctgcgtggtggtggatgtgtctcacgaggaccccgaagtgaagttcaattggtacgtggacggcgtggaagtgcacaacgccaagaccaagcctagagaggaacagtacaactccacctacagagtggtgtccgtgctgaccgtgctgcaccaggattggctgaacggcaaagagtacaagtgcaaggtgtccaacaaggccctgcctgctcctatcgaaaagaccatctccaaggccaagggccagcctagggaaccccaggtttacacactgcctccatctcgggacgagctgaccaagaatcaggtgtccctgacctgtctggtcaagggcttctacccttccgatatcgccgtggaatgggagagcaatggccagcctgagaacaactacaagacaacccctcctgtgctggactccgacggctcattcttcctgtatagcaagctgacagtggacaagtcccggtggcagcagggcaacgtgttctcctgttctgtgatgcacgaggccctgcacaaccactacacccagaagagtctgtccttgagcccgggc

SEQ ID NO: 71 - DNA, 1923 bp, Artificial Sequence
  Fusion protein_DNA sequence_GIC-1114
cggtctaagcagagaaggcctcagggcctgcctaacaataccgcctcctggtttaccgctctgacccagcacggcaaagaggacctgaagttccctagaggacagggcgtgcccatcaacaccaactctagccctgacgaccagatcggctactacagacgggccaccagaagaatcagaggcggcgacggcaagatgaaggacctgtctcctcggtggtacttctactacctcggcaccggaccagaggctggattgccttatggcgccaacaaggacggcatcatctgggttgcaacagagggcgctctgaacacccctaaggaccacatcggcacccggaatcctgccaacaatgctgccattgtgctgcagctgccacagggcacaacactgcctaagggcttttacgccgagggctctagaggcggctctcaggcctcttccagatcctccagtagatcacgtggcggcggaggatccggcggtggtggttccggcggaggcggttctgaacctaagtcctccgacaagacccacacctgtcctccatgtcctgctccagaactgctcggcggaccttccgtgtttctgttcccacctaagccaaaggacaccctgatgatcagcagaacccctgaagtgacctgcgtggtggtggatgtgtctcacgaggaccccgaagtgaagttcaattggtacgtggacggcgtggaagtgcacaacgccaagaccaagcctagagaggaacagtacaactccacctacagagtggtgtccgtgctgaccgtgctgcaccaggattggctgaacggcaaagagtacaagtgcaaggtgtccaacaaggccctgcctgctcctatcgaaaagaccatctccaaggccaagggccagcctagggaaccccaggtttacacactgcctccatctcgggacgagctgaccaagaatcaggtgtccctgacctgtctggtcaagggcttctacccttccgatatcgccgtggaatgggagagcaatggccagcctgagaacaactacaagacaacccctcctgtgctggactccgacggctcattcttcctgtatagcaagctgacagtggacaagtcccggtggcagcagggcaacgtgttctcctgttctgtgatgcacgaggccctgcacaaccactacacccagaagagtctgtccttgagcccgggcggtggcggtggaagcggaggtggcggatctggtggcggaggtagtggcggaggcggatctagagttcagcctaccgagtccatcgtgcggttccccaacatcaccaacctgtgtcctttcggcgaggtgttcaacgctaccagattcgcctctgtgtacgcctggaaccggaagcggatctctaactgcgtggccgactactccgtgctgtacaactctgcctccttcagcaccttcaagtgctacggcgtgtcccctaccaagctgaacgacctgtgcttcaccaacgtgtacgccgactccttcgtgatcaggggcgacgaagttcggcagatcgctcctggacagaccggcaagatcgccgactacaattacaagctgcccgacgacttcaccggctgcgtgatcgcttggaactccaacaacctggactccaaagtcggcggcaactacaactacctgtaccggctgttccggaagtccaacctgaagcctttcgagcgggacatctccaccgagatctaccaggctggcagcaccccttgcaatggcgtcgagggcttcaactgctacttcccactgcagtcctacggcttccagcctaccaatggcgtgggctaccagccttatagagtggtggtgctgtccttcgagctgctgcatgctcctgctaccgtgtgcggccctaagaaatctaccaacctggtcaagaacaag

SEQ ID NO: 72 - DNA, 1923 bp, Artificial Sequence
  Fusion protein_DNA sequence_GIC-1114m(L137A, F168A)
cggtctaagcagagaaggcctcagggcctgcctaacaataccgcctcctggtttaccgctctgacccagcacggcaaagaggacctgaagttccctagaggacagggcgtgcccatcaacaccaactctagccctgacgaccagatcggctactacagacgggccaccagaagaatcagaggcggcgacggcaagatgaaggacctgtctcctcggtggtacttctactacctcggcaccggaccagaggctggattgccttatggcgccaacaaggacggcatcatctgggttgcaacagagggcgctctgaacacccctaaggaccacatcggcacccggaatcctgccaacaatgctgccattgtgctgcagctgccacagggcacaacactgcctaagggcttttacgccgagggctctagaggcggctctcaggcctcttccagatcctccagtagatcacgtggcggcggaggatccggtggtggtggatctggtggcggaggctctgaacctaagtcctccgacaagacccacacctgtcctccatgtcctgctccagaactgctcggcggaccttccgtgtttctgttccctccaaagcctaaggacaccctgatgatctctcggacccctgaagtgacctgcgtggtggtcgatgtgtctcacgaggacccagaagtgaagttcaattggtacgtggacggcgtggaagtgcacaacgccaagaccaagcctagagaggaacagtacaactccacctacagagtggtgtccgtgctgaccgtgctgcaccaggattggctgaatggcaaagagtacaagtgcaaggtgtccaacaaggccctgcctgctcctatcgaaaagaccatctccaaggccaagggccagcctagggaaccccaggtttacaccttgcctccatctcgggacgagctgaccaagaaccaggtgtccctgacctgtctggtcaagggcttctacccctccgatatcgccgtggaatgggagtctaatggccagcctgagaacaactacaagacaacccctcctgtgctggactccgacggctcattcttcctgtactccaagctgacagtggacaagtccagatggcagcagggcaacgtgttctcctgctccgtgatgcacgaggccctgcacaatcactacacacagaagtccctgtctctgtcccctggtggtggcggcggttcaggcggcggtggaagtggcggtggcggatctggcggaggtggtagtagagtgcagcctaccgagtccatcgtgcggttccccaacatcaccaacctgtgtcctttcggcgaggtgttcaacgctaccagattcgcctctgtgtacgcctggaaccggaagcggatctctaactgcgtggccgactactccgtgctgtacaactctgcctccttcagcaccttcaagtgctacggcgtgtcccctaccaagctgaacgacctgtgcttcaccaacgtgtacgccgactccttcgtgatcaggggcgacgaagttcggcagatcgctcctggacagaccggcaagatcgccgactacaattacaagctgcccgacgacttcaccggctgcgtgatcgcttggaactccaacaacctggactccaaagtcggcggcaactacaactacctgtaccgggccttcagaaagtccaacctgaagcctttcgagcgggacatctccaccgagatctaccaggctggcagcaccccttgcaatggcgttgaaggcgccaactgctacttcccactgcagtcctacggcttccagcctaccaatggcgtgggctaccagccttatagagtggtggtgctgtccttcgagctgctgcatgctcctgctacagtgtgcggccccaagaaatctaccaacctggtcaagaacaag

SEQ ID NO: 73 - DNA, 1923 bp, Artificial Sequence
  Fusion protein_DNA sequence_GIC-1114m(L137A)
cggtctaagcagagaaggcctcagggcctgcctaacaataccgcctcctggtttaccgctctgacccagcacggcaaagaggacctgaagttccctagaggacagggcgtgcccatcaacaccaactctagccctgacgaccagatcggctactacagacgggccaccagaagaatcagaggcggcgacggcaagatgaaggacctgtctcctcggtggtacttctactacctcggcaccggaccagaggctggattgccttatggcgccaacaaggacggcatcatctgggttgcaacagagggcgctctgaacacccctaaggaccacatcggcacccggaatcctgccaacaatgctgccattgtgctgcagctgccacagggcacaacactgcctaagggcttttacgccgagggctctagaggcggctctcaggcctcttccagatcctccagtagatcacgtggcggcggaggatccggtggtggtggatctggtggcggaggctctgaacctaagtcctccgacaagacccacacctgtcctccatgtcctgctccagaactgctcggcggaccttccgtgtttctgttccctccaaagcctaaggacaccctgatgatctctcggacccctgaagtgacctgcgtggtggtcgatgtgtctcacgaggacccagaagtgaagttcaattggtacgtggacggcgtggaagtgcacaacgccaagaccaagcctagagaggaacagtacaactccacctacagagtggtgtccgtgctgaccgtgctgcaccaggattggctgaatggcaaagagtacaagtgcaaggtgtccaacaaggccctgcctgctcctatcgaaaagaccatctccaaggccaagggccagcctagggaaccccaggtttacaccttgcctccatctcgggacgagctgaccaagaaccaggtgtccctgacctgtctggtcaagggcttctacccctccgatatcgccgtggaatgggagtctaatggccagcctgagaacaactacaagacaacccctcctgtgctggactccgacggctcattcttcctgtactccaagctgacagtggacaagtccagatggcagcagggcaacgtgttctcctgctccgtgatgcacgaggccctgcacaatcactacacacagaagtccctgtctctgtcccctggtggtggcggcggttcaggcggcggtggaagtggcggtggcggatctggcggaggtggtagtagagtgcagcctaccgagtccatcgtgcggttccccaacatcaccaacctgtgtcctttcggcgaggtgttcaacgctaccagattcgcctctgtgtacgcctggaaccggaagcggatctctaactgcgtggccgactactccgtgctgtacaactctgcctccttcagcaccttcaagtgctacggcgtgtcccctaccaagctgaacgacctgtgcttcaccaacgtgtacgccgactccttcgtgatcaggggcgacgaagttcggcagatcgctcctggacagaccggcaagatcgccgactacaattacaagctgcccgacgacttcaccggctgcgtgatcgcttggaactccaacaacctggactccaaagtcggcggcaactacaactacctgtaccgggccttcagaaagtccaacctgaagcctttcgagcgggacatctccaccgagatctaccaggctggcagcaccccttgcaatggcgttgaaggcttcaactgctacttcccactgcagtcctacggcttccagcctaccaatggcgtgggctaccagccttatagagtggtggtgctgtccttcgagctgctgcatgctcctgctacagtgtgcggccccaagaaatctaccaacctggtcaagaacaag

SEQ ID NO: 74 - DNA, 1923 bp, Artificial Sequence
  Fusion protein_DNA sequence_GIC-1114m(F168A)
cggtctaagcagagaaggcctcagggcctgcctaacaataccgcctcctggtttaccgctctgacccagcacggcaaagaggacctgaagttccctagaggacagggcgtgcccatcaacaccaactctagccctgacgaccagatcggctactacagacgggccaccagaagaatcagaggcggcgacggcaagatgaaggacctgtctcctcggtggtacttctactacctcggcaccggaccagaggctggattgccttatggcgccaacaaggacggcatcatctgggttgcaacagagggcgctctgaacacccctaaggaccacatcggcacccggaatcctgccaacaatgctgccattgtgctgcagctgccacagggcacaacactgcctaagggcttttacgccgagggctctagaggcggctctcaggcctcttccagatcctccagtagatcacgtggcggcggaggatccggtggtggtggatctggtggcggaggctctgaacctaagtcctccgacaagacccacacctgtcctccatgtcctgctccagaactgctcggcggaccttccgtgtttctgttccctccaaagcctaaggacaccctgatgatctctcggacccctgaagtgacctgcgtggtggtcgatgtgtctcacgaggacccagaagtgaagttcaattggtacgtggacggcgtggaagtgcacaacgccaagaccaagcctagagaggaacagtacaactccacctacagagtggtgtccgtgctgaccgtgctgcaccaggattggctgaatggcaaagagtacaagtgcaaggtgtccaacaaggccctgcctgctcctatcgaaaagaccatctccaaggccaagggccagcctagggaaccccaggtttacaccttgcctccatctcgggacgagctgaccaagaaccaggtgtccctgacctgtctggtcaagggcttctacccctccgatatcgccgtggaatgggagtctaatggccagcctgagaacaactacaagacaacccctcctgtgctggactccgacggctcattcttcctgtactccaagctgacagtggacaagtccagatggcagcagggcaacgtgttctcctgctccgtgatgcacgaggccctgcacaatcactacacacagaagtccctgtctctgtcccctggtggtggcggcggttcaggcggcggtggaagtggcggtggcggatctggcggaggtggtagtagagtgcagcctaccgagtccatcgtgcggttccccaacatcaccaacctgtgtcctttcggcgaggtgttcaacgctaccagattcgcctctgtgtacgcctggaaccggaagcggatctctaactgcgtggccgactactccgtgctgtacaactctgcctccttcagcaccttcaagtgctacggcgtgtcccctaccaagctgaacgacctgtgcttcaccaacgtgtacgccgactccttcgtgatcaggggcgacgaagttcggcagatcgctcctggacagaccggcaagatcgccgactacaattacaagctgcccgacgacttcaccggctgcgtgatcgcttggaactccaacaacctggactccaaagtcggcggcaactacaactacctgtaccggctgttcagaaagtccaacctgaagcctttcgagcgggacatctccaccgagatctaccaggctggcagcaccccttgcaatggcgttgaaggcgccaactgctacttcccactgcagtcctacggcttccagcctaccaatggcgtgggctaccagccttatagagtggtggtgctgtccttcgagctgctgcatgctcctgctacagtgtgcggccccaagaaatctaccaacctggtcaagaacaag

SEQ ID NO: 75 - DNA, 1923 bp, Artificial Sequence
  Fusion protein_DNA sequence_GIC-1114m(G184D)
cggtctaagcagagaaggcctcagggcctgcctaacaataccgcctcctggtttaccgctctgacccagcacggcaaagaggacctgaagttccctagaggacagggcgtgcccatcaacaccaactctagccctgacgaccagatcggctactacagacgggccaccagaagaatcagaggcggcgacggcaagatgaaggacctgtctcctcggtggtacttctactacctcggcaccggaccagaggctggattgccttatggcgccaacaaggacggcatcatctgggttgcaacagagggcgctctgaacacccctaaggaccacatcggcacccggaatcctgccaacaatgctgccattgtgctgcagctgccacagggcacaacactgcctaagggcttttacgccgagggctctagaggcggctctcaggcctcttccagatcctccagtagatcacgtggcggcggaggatccggtggtggtggatctggtggcggaggctctgaacctaagtcctccgacaagacccacacctgtcctccatgtcctgctccagaactgctcggcggaccttccgtgtttctgttccctccaaagcctaaggacaccctgatgatctctcggacccctgaagtgacctgcgtggtggtcgatgtgtctcacgaggacccagaagtgaagttcaattggtacgtggacggcgtggaagtgcacaacgccaagaccaagcctagagaggaacagtacaactccacctacagagtggtgtccgtgctgaccgtgctgcaccaggattggctgaatggcaaagagtacaagtgcaaggtgtccaacaaggccctgcctgctcctatcgaaaagaccatctccaaggccaagggccagcctagggaaccccaggtttacaccttgcctccatctcgggacgagctgaccaagaaccaggtgtccctgacctgtctggtcaagggcttctacccctccgatatcgccgtggaatgggagtctaatggccagcctgagaacaactacaagacaacccctcctgtgctggactccgacggctcattcttcctgtactccaagctgacagtggacaagtccagatggcagcagggcaacgtgttctcctgctccgtgatgcacgaggccctgcacaatcactacacacagaagtccctgtctctgtcccctggtggtggcggcggttcaggcggcggtggaagtggcggtggcggatctggcggaggtggtagtagagttcagcctaccgagtccatcgtgcggttccccaacatcaccaacctgtgtcctttcggcgaggtgttcaacgctaccagattcgcctctgtgtacgcctggaaccggaagcggatctctaactgcgtggccgactactccgtgctgtacaactctgcctccttcagcaccttcaagtgctacggcgtgtcccctaccaagctgaacgacctgtgcttcaccaacgtgtacgccgactccttcgtgatcaggggcgacgaagttcggcagatcgctcctggacagaccggcaagatcgccgactacaattacaagctgcccgacgacttcaccggctgcgtgatcgcttggaactccaacaacctggactccaaagtcggcggcaactacaactacctgtaccggctgttccggaagtccaacctgaagcctttcgagcgggacatctccaccgagatctaccaggctggcagcaccccttgcaatggcgtcgagggcttcaactgctacttcccactgcagtcctacggcttccagcctaccaatgacgtgggctaccagccttatagagtggtggtgctgtccttcgagctgctgcatgctcctgctaccgtgtgcggccctaagaaatctaccaacctggtcaagaacaag

SEQ ID NO: 76 - DNA, 1923 bp, Artificial Sequence
  Fusion protein_DNA sequence_GIC-1114m(L137A, G164A, V165A, F168A, Q175A, S176A, N183A)
cggtctaagcagagaaggcctcagggcctgcctaacaataccgcctcctggtttaccgctctgacccagcacggcaaagaggacctgaagttccctagaggacagggcgtgcccatcaacaccaactctagccctgacgaccagatcggctactacagacgggccaccagaagaatcagaggcggcgacggcaagatgaaggacctgtctcctcggtggtacttctactacctcggcaccggaccagaggctggattgccttatggcgccaacaaggacggcatcatctgggttgcaacagagggcgctctgaacacccctaaggaccacatcggcacccggaatcctgccaacaatgctgccattgtgctgcagctgccacagggcacaacactgcctaagggcttttacgccgagggctctagaggcggctctcaggcctcttccagatcctccagtagatcacgtggcggcggaggatccggtggtggtggatctggtggcggaggctctgaacctaagtcctccgacaagacccacacctgtcctccatgtcctgctccagaactgctcggcggaccttccgtgtttctgttccctccaaagcctaaggacaccctgatgatctctcggacccctgaagtgacctgcgtggtggtcgatgtgtctcacgaggacccagaagtgaagttcaattggtacgtggacggcgtggaagtgcacaacgccaagaccaagcctagagaggaacagtacaactccacctacagagtggtgtccgtgctgaccgtgctgcaccaggattggctgaatggcaaagagtacaagtgcaaggtgtccaacaaggccctgcctgctcctatcgaaaagaccatctccaaggccaagggccagcctagggaaccccaggtttacaccttgcctccatctcgggacgagctgaccaagaaccaggtgtccctgacctgtctggtcaagggcttctacccctccgatatcgccgtggaatgggagtctaatggccagcctgagaacaactacaagacaacccctcctgtgctggactccgacggctcattcttcctgtactccaagctgacagtggacaagtccagatggcagcagggcaacgtgttctcctgctccgtgatgcacgaggccctgcacaatcactacacacagaagtccctgtctctgtcccctggtggtggcggcggttcaggcggcggtggaagtggcggtggcggatctggcggaggtggtagtagagtgcagcctaccgagtctatcgtgcggttccccaacatcaccaacctgtgtcctttcggcgaggtgttcaacgccaccagattcgcctctgtgtacgcctggaaccggaagcggatctctaactgcgtggccgactactccgtgctgtacaactccgcctccttcagcaccttcaagtgctacggcgtgtcccctaccaagctgaacgacctgtgcttcaccaacgtgtacgccgactccttcgtgatcagaggcgacgaagtgcggcagatcgctcctggacagaccggcaagatcgccgactacaactacaagctgcccgacgacttcaccggctgtgtgatcgcttggaactccaacaacctggactccaaagtcggcggcaactacaattacctgtaccgggccttccgcaagtccaacctgaagcctttcgagcgggacatctccaccgagatctaccaggctggcagcaccccttgtaatgctgccgaaggcgccaactgctactttcctctggccgcctatggcttccagcctacagctggcgttggctaccagccttatagagtggtggtgctgtccttcgagctgctgcatgctcctgctaccgtgtgcggccctaagaaatctaccaacctggtcaagaacaaa

SEQ ID NO: 77 - DNA, 1923 bp, Artificial Sequence
  Fusion protein_DNA sequence_GIC-1114N
agagttcagcctaccgagtccatcgtgcggttccccaacatcaccaacctgtgtcctttcggcgaggtgttcaacgctaccagattcgcctctgtgtacgcctggaaccggaagcggatctctaactgcgtggccgactactccgtgctgtacaactctgcctccttcagcaccttcaagtgctacggcgtgtcccctaccaagctgaacgacctgtgcttcaccaacgtgtacgccgactccttcgtgatcaggggcgacgaagttcggcagatcgctcctggacagaccggcaagatcgccgactacaattacaagctgcccgacgacttcaccggctgcgtgatcgcttggaactccaacaacctggactccaaagtcggcggcaactacaactacctgtaccggctgttccggaagtccaacctgaagcctttcgagcgggacatctccaccgagatctaccaggctggcagcaccccttgcaatggcgtcgagggcttcaactgctacttcccactgcagtcctacggcttccagcctaccaatggcgtgggctaccagccttatagagtggtggtgctgtccttcgagctgctgcatgctcctgctaccgtgtgcggccctaagaaatctaccaacctggtcaagaacaagggcggcggaggatccggcggtggtggttccggcggaggcggttctgaacctaagtcctccgacaagacccacacctgtcctccatgtcctgctccagaactgctcggcggaccttccgtgtttctgttcccacctaagccaaaggacaccctgatgatcagcagaacccctgaagtgacctgcgtggtggtggatgtgtctcacgaggaccccgaagtgaagttcaattggtacgtggacggcgtggaagtgcacaacgccaagaccaagcctagagaggaacagtacaactccacctacagagtggtgtccgtgctgaccgtgctgcaccaggattggctgaacggcaaagagtacaagtgcaaggtgtccaacaaggccctgcctgctcctatcgaaaagaccatctccaaggccaagggccagcctagggaaccccaggtttacacactgcctccatctcgggacgagctgaccaagaatcaggtgtccctgacctgtctggtcaagggcttctacccttccgatatcgccgtggaatgggagagcaatggccagcctgagaacaactacaagacaacccctcctgtgctggactccgacggctcattcttcctgtatagcaagctgacagtggacaagtcccggtggcagcagggcaacgtgttctcctgttctgtgatgcacgaggccctgcacaaccactacacccagaagagtctgtccttgagcccgggcggtggcggtggaagcggaggtggcggatctggtggcggaggtagtggcggaggcggatctcggtctaagcagagaaggcctcagggcctgcctaacaataccgcctcctggtttaccgctctgacccagcacggcaaagaggacctgaagttccctagaggacagggcgtgcccatcaacaccaactctagccctgacgaccagatcggctactacagacgggccaccagaagaatcagaggcggcgacggcaagatgaaggacctgtctcctcggtggtacttctactacctcggcaccggaccagaggctggattgccttatggcgccaacaaggacggcatcatctgggttgcaacagagggcgctctgaacacccctaaggaccacatcggcacccggaatcctgccaacaatgctgccattgtgctgcagctgccacagggcacaacactgcctaagggcttttacgccgagggctctagaggcggctctcaggcctcttccagatcctccagtagatcacgt

SEQ ID NO: 78 - DNA, 1923 bp, Artificial Sequence
  Fusion protein_DNA sequence_GIC-1114Nm(L137A, F168A)
agagtgcagcctaccgagtccatcgtgcggttccccaacatcaccaacctgtgtcctttcggcgaggtgttcaacgctaccagattcgcctctgtgtacgcctggaaccggaagcggatctctaactgcgtggccgactactccgtgctgtacaactctgcctccttcagcaccttcaagtgctacggcgtgtcccctaccaagctgaacgacctgtgcttcaccaacgtgtacgccgactccttcgtgatcaggggcgacgaagttcggcagatcgctcctggacagaccggcaagatcgccgactacaattacaagctgcccgacgacttcaccggctgcgtgatcgcttggaactccaacaacctggactccaaagtcggcggcaactacaactacctgtaccgggccttcagaaagtccaacctgaagcctttcgagcgggacatctccaccgagatctaccaggctggcagcaccccttgcaatggcgttgaaggcgccaactgctacttcccactgcagtcctacggcttccagcctaccaatggcgtgggctaccagccttatagagtggtggtgctgtccttcgagctgctgcatgctcctgctacagtgtgcggccccaagaaatctaccaacctggtcaagaacaagggcggcggaggatccggtggtggtggatctggtggcggaggctctgaacctaagtcctccgacaagacccacacctgtcctccatgtcctgctccagaactgctcggcggaccttccgtgtttctgttccctccaaagcctaaggacaccctgatgatctctcggacccctgaagtgacctgcgtggtggtcgatgtgtctcacgaggacccagaagtgaagttcaattggtacgtggacggcgtggaagtgcacaacgccaagaccaagcctagagaggaacagtacaactccacctacagagtggtgtccgtgctgaccgtgctgcaccaggattggctgaatggcaaagagtacaagtgcaaggtgtccaacaaggccctgcctgctcctatcgaaaagaccatctccaaggccaagggccagcctagggaaccccaggtttacaccttgcctccatctcgggacgagctgaccaagaaccaggtgtccctgacctgtctggtcaagggcttctacccctccgatatcgccgtggaatgggagtctaatggccagcctgagaacaactacaagacaacccctcctgtgctggactccgacggctcattcttcctgtactccaagctgacagtggacaagtccagatggcagcagggcaacgtgttctcctgctccgtgatgcacgaggccctgcacaatcactacacacagaagtccctgtctctgtcccctggtggtggcggcggttcaggcggcggtggaagtggcggtggcggatctggcggaggtggtagtcggtctaagcagagaaggcctcagggcctgcctaacaataccgcctcctggtttaccgctctgacccagcacggcaaagaggacctgaagttccctagaggacagggcgtgcccatcaacaccaactctagccctgacgaccagatcggctactacagacgggccaccagaagaatcagaggcggcgacggcaagatgaaggacctgtctcctcggtggtacttctactacctcggcaccggaccagaggctggattgccttatggcgccaacaaggacggcatcatctgggttgcaacagagggcgctctgaacacccctaaggaccacatcggcacccggaatcctgccaacaatgctgccattgtgctgcagctgccacagggcacaacactgcctaagggcttttacgccgagggctctagaggcggctctcaggcctcttccagatcctccagtagatcacgt

SEQ ID NO: 79 - DNA, 2319 bp, Artificial Sequence
  Fusion protein_DNA sequence_GIC-1132m(L137A, F168A)
cggctgttcgcccggaccagatctatgtggtctttcaaccccgagacaaacatcctgctgaacgtgccactgcacggcaccatcctgaccagacctctgctggaatccgagctggtcatcggcgctgtgatcctgagaggccacctgagaatcgctggccaccatctgggcagatgcgacatcaaggacctgcctaaagagatcaccgtcgccacctctcggaccctgagctactataagctgggcgcctctcagagagtggctggcgattctggctttgccgcctactccagataccggatcggcaactacaagctgaacaccgaccactcctccagctccgacaatatcgctctgctggtgcagggcggaggcggatctggtggcggaggatctcggtctaagcagagaaggcctcagggcctgcctaacaataccgcctcctggtttaccgctctgacccagcacggcaaagaggacctgaagttccctagaggacagggcgtgcccatcaacaccaactctagccctgacgaccagatcggctactacagacgggccaccagaagaatcagaggcggcgacggcaagatgaaggacctgtctcctcggtggtacttctactacctcggcaccggaccagaggctggattgccttatggcgccaacaaggacggcatcatctgggttgcaacagagggcgctctgaacacccctaaggaccacatcggcacccggaatcctgccaacaatgctgccattgtgctgcagctgccacagggcacaacactgcctaagggcttttacgccgagggctctagaggcggctctcaggcctcttccagatcctccagtagatcacgtggcggcggaggatccggtggtggtggatctggtggcggaggctctgaacctaagtcctccgacaagacccacacctgtcctccatgtcctgctccagaactgctcggcggaccttccgtgtttctgttccctccaaagcctaaggacaccctgatgatctctcggacccctgaagtgacctgcgtggtggtcgatgtgtctcacgaggacccagaagtgaagttcaattggtacgtggacggcgtggaagtgcacaacgccaagaccaagcctagagaggaacagtacaactccacctacagagtggtgtccgtgctgaccgtgctgcaccaggattggctgaatggcaaagagtacaagtgcaaggtgtccaacaaggccctgcctgctcctatcgaaaagaccatctccaaggccaagggccagcctagggaaccccaggtttacaccttgcctccatctcgggacgagctgaccaagaaccaggtgtccctgacctgtctggtcaagggcttctacccctccgatatcgccgtggaatgggagtctaatggccagcctgagaacaactacaagacaacccctcctgtgctggactccgacggctcattcttcctgtactccaagctgacagtggacaagtccagatggcagcagggcaacgtgttctcctgctccgtgatgcacgaggccctgcacaatcactacacacagaagtccctgtctctgtcccctggtggtggcggcggttcaggcggcggtggaagtggcggtggcggatctggcggaggtggtagtagagtgcagcctaccgagtccatcgtgcggttccccaacatcaccaacctgtgtcctttcggcgaggtgttcaacgctaccagattcgcctctgtgtacgcctggaaccggaagcggatctctaactgcgtggccgactactccgtgctgtacaactctgcctccttcagcaccttcaagtgctacggcgtgtcccctaccaagctgaacgacctgtgcttcaccaacgtgtacgccgactccttcgtgatcaggggcgacgaagttcggcagatcgctcctggacagaccggcaagatcgccgactacaattacaagctgcccgacgacttcaccggctgcgtgatcgcttggaactccaacaacctggactccaaagtcggcggcaactacaactacctgtaccgggccttcagaaagtccaacctgaagcctttcgagcgggacatctccaccgagatctaccaggctggcagcaccccttgcaatggcgttgaaggcgccaactgctacttcccactgcagtcctacggcttccagcctaccaatggcgtgggctaccagccttatagagtggtggtgctgtccttcgagctgctgcatgctcctgctacagtgtgcggccccaagaaatctaccaacctggtcaagaacaag

SEQ ID NO: 80 - DNA, 2319 bp, Artificial Sequence
  Fusion protein_DNA sequence_GIC-1133m(L137A, F168A)
cggtctaagcagagaaggcctcagggcctgcctaacaataccgcctcctggtttaccgctctgacccagcacggcaaagaggacctgaagttccctagaggacagggcgtgcccatcaacaccaactctagccctgacgaccagatcggctactacagacgggccaccagaagaatcagaggcggcgacggcaagatgaaggacctgtctcctcggtggtacttctactacctcggcaccggaccagaggctggattgccttatggcgccaacaaggacggcatcatctgggttgcaacagagggcgctctgaacacccctaaggaccacatcggcacccggaatcctgccaacaatgctgccattgtgctgcagctgccacagggcacaacactgcctaagggcttttacgccgagggctctagaggcggctctcaggcctcttccagatcctccagtagatcacgtggcggaggcggatctggtggcggaggatctcggctgttcgcccggaccagatctatgtggtctttcaaccccgagacaaacatcctgctgaacgtgccactgcacggcaccatcctgaccagacctctgctggaatccgagctggtcatcggcgctgtgatcctgagaggccacctgagaatcgctggccaccatctgggcagatgcgacatcaaggacctgcctaaagagatcaccgtcgccacctctcggaccctgagctactataagctgggcgcctctcagagagtggctggcgattctggctttgccgcctactccagataccggatcggcaactacaagctgaacaccgaccactcctccagctccgacaatatcgctctgctggtgcagggcggcggaggatccggtggtggtggatctggtggcggaggctctgaacctaagtcctccgacaagacccacacctgtcctccatgtcctgctccagaactgctcggcggaccttccgtgtttctgttccctccaaagcctaaggacaccctgatgatctctcggacccctgaagtgacctgcgtggtggtcgatgtgtctcacgaggacccagaagtgaagttcaattggtacgtggacggcgtggaagtgcacaacgccaagaccaagcctagagaggaacagtacaactccacctacagagtggtgtccgtgctgaccgtgctgcaccaggattggctgaatggcaaagagtacaagtgcaaggtgtccaacaaggccctgcctgctcctatcgaaaagaccatctccaaggccaagggccagcctagggaaccccaggtttacaccttgcctccatctcgggacgagctgaccaagaaccaggtgtccctgacctgtctggtcaagggcttctacccctccgatatcgccgtggaatgggagtctaatggccagcctgagaacaactacaagacaacccctcctgtgctggactccgacggctcattcttcctgtactccaagctgacagtggacaagtccagatggcagcagggcaacgtgttctcctgctccgtgatgcacgaggccctgcacaatcactacacacagaagtccctgtctctgtcccctggtggtggcggcggttcaggcggcggtggaagtggcggtggcggatctggcggaggtggtagtagagtgcagcctaccgagtccatcgtgcggttccccaacatcaccaacctgtgtcctttcggcgaggtgttcaacgctaccagattcgcctctgtgtacgcctggaaccggaagcggatctctaactgcgtggccgactactccgtgctgtacaactctgcctccttcagcaccttcaagtgctacggcgtgtcccctaccaagctgaacgacctgtgcttcaccaacgtgtacgccgactccttcgtgatcaggggcgacgaagttcggcagatcgctcctggacagaccggcaagatcgccgactacaattacaagctgcccgacgacttcaccggctgcgtgatcgcttggaactccaacaacctggactccaaagtcggcggcaactacaactacctgtaccgggccttcagaaagtccaacctgaagcctttcgagcgggacatctccaccgagatctaccaggctggcagcaccccttgcaatggcgttgaaggcgccaactgctacttcccactgcagtcctacggcttccagcctaccaatggcgtgggctaccagccttatagagtggtggtgctgtccttcgagctgctgcatgctcctgctacagtgtgcggccccaagaaatctaccaacctggtcaagaacaag

SEQ ID NO: 81 - DNA, 2340 bp, Artificial Sequence
  Fusion protein_DNA sequence_GIC-1151
agagtgcagcctaccgagtccatcgtgcggttccccaacatcaccaacctgtgtcctttcggcgaggtgttcaacgctaccagattcgcctctgtgtacgcctggaaccggaagcggatctctaactgcgtggccgactactccgtgctgtacaactctgcctccttcagcaccttcaagtgctacggcgtgtcccctaccaagctgaacgacctgtgcttcaccaacgtgtacgccgactccttcgtgatcaggggcgacgaagttcggcagatcgctcctggacagaccggcaagatcgccgactacaattacaagctgcccgacgacttcaccggctgcgtgatcgcttggaactccaacaacctggactccaaagtcggcggcaactacaactacctgtaccggctgttcagaaagtccaacctgaagcctttcgagcgggacatctccaccgagatctaccaggctggcagcaccccttgcaatggcgttgaaggcttcaactgctacttcccactgcagtcctacggcttccagcctaccaatggcgtgggctaccagccttatagagtggtggtgctgtccttcgagctgctgcatgctcctgctacagtgtgcggccccaagaaatctaccaacctggtcaagaacaagggtggcagtggtggctctggcggatctcggtctaagcagagaaggcctcagggcctgcctaacaataccgcctcctggtttaccgctctgacccagcacggcaaagaggacctgaagttccctagaggacagggcgtgcccatcaacaccaactctagccctgacgaccagatcggctactacagacgggccaccagaagaatcagaggcggcgacggcaagatgaaggacctgtctcctcggtggtacttctactacctcggcaccggaccagaggctggattgccttatggcgccaacaaggacggcatcatctgggttgcaacagagggcgctctgaacacccctaaggaccacatcggcacccggaatcctgccaacaatgctgccattgtgctgcagctgccacagggcacaacactgcctaagggcttttacgccgagggctctagaggcggctctcaggcctcttccagatcctccagtagatcacgtggcggatccggaggatcaggtggaagcggaggttcacggtctaagcagagaaggcctcagggcctgcctaacaataccgcctcctggtttaccgctctgacccagcacggcaaagaggacctgaagttccctagaggacagggcgtgcccatcaacaccaactctagccctgacgaccagatcggctactacagacgggccaccagaagaatcagaggcggcgacggcaagatgaaggacctgtctcctcggtggtacttctactacctcggcaccggaccagaggctggattgccttatggcgccaacaaggacggcatcatctgggttgcaacagagggcgctctgaacacccctaaggaccacatcggcacccggaatcctgccaacaatgctgccattgtgctgcagctgccacagggcacaacactgcctaagggcttttacgccgagggctctagaggcggctctcaggcctcttccagatcctccagtagatcacgtggtggtagtggcggaagcggcggctccagagttcagcctaccgagtccatcgtgcggttccccaacatcaccaacctgtgtcctttcggcgaggtgttcaacgctaccagattcgcctctgtgtacgcctggaaccggaagcggatctctaactgcgtggccgactactccgtgctgtacaactctgcctccttcagcaccttcaagtgctacggcgtgtcccctaccaagctgaacgacctgtgcttcaccaacgtgtacgccgactccttcgtgatcaggggcgacgaagttcggcagatcgcacctggccagaccggcaagatcgccgactataactacaagctgcccgacgacttcaccggctgtgtgatcgcttggaactccaacaacctggactccaaagtcggcggcaactacaactacctgtaccggctgttccggaagtccaacctgaagcctttcgagcgggacatctccaccgagatctaccaggctggctctaccccttgcaatggcgtcgagggcttcaactgctacttcccactgcagtcctacggcttccagcctaccaatggcgtgggctaccagccttatagagtggtggtgctgtccttcgagctgctgcatgctcctgctaccgtgtgcggccctaagaaatctaccaacctggtcaagaacaag

SEQ ID NO: 82 - DNA, 2340 bp, Artificial Sequence
  Fusion protein_DNA sequence_GIC-1151m(L137A, F168A)
agagtgcagcctaccgagtccatcgtgcggttccccaacatcaccaacctgtgtcctttcggcgaggtgttcaacgctaccagattcgcctctgtgtacgcctggaaccggaagcggatctctaactgcgtggccgactactccgtgctgtacaactctgcctccttcagcaccttcaagtgctacggcgtgtcccctaccaagctgaacgacctgtgcttcaccaacgtgtacgccgactccttcgtgatcaggggcgacgaagttcggcagatcgctcctggacagaccggcaagatcgccgactacaattacaagctgcccgacgacttcaccggctgcgtgatcgcttggaactccaacaacctggactccaaagtcggcggcaactacaactacctgtaccgggccttcagaaagtccaacctgaagcctttcgagcgggacatctccaccgagatctaccaggctggcagcaccccttgcaatggcgttgaaggcgccaactgctacttcccactgcagtcctacggcttccagcctaccaatggcgtgggctaccagccttatagagtggtggtgctgtccttcgagctgctgcatgctcctgctacagtgtgcggccccaagaaatctaccaacctggtcaagaacaagggtggcagtggtggctctggcggatctcggtctaagcagagaaggcctcagggcctgcctaacaataccgcctcctggtttaccgctctgacccagcacggcaaagaggacctgaagttccctagaggacagggcgtgcccatcaacaccaactctagccctgacgaccagatcggctactacagacgggccaccagaagaatcagaggcggcgacggcaagatgaaggacctgtctcctcggtggtacttctactacctcggcaccggaccagaggctggattgccttatggcgccaacaaggacggcatcatctgggttgcaacagagggcgctctgaacacccctaaggaccacatcggcacccggaatcctgccaacaatgctgccattgtgctgcagctgccacagggcacaacactgcctaagggcttttacgccgagggctctagaggcggctctcaggcctcttccagatcctccagtagatcacgtggcggatccggaggatcaggtggaagcggaggttcacggtctaagcagagaaggcctcagggcctgcctaacaataccgcctcctggtttaccgctctgacccagcacggcaaagaggacctgaagttccctagaggacagggcgtgcccatcaacaccaactctagccctgacgaccagatcggctactacagacgggccaccagaagaatcagaggcggcgacggcaagatgaaggacctgtctcctcggtggtacttctactacctcggcaccggaccagaggctggattgccttatggcgccaacaaggacggcatcatctgggttgcaacagagggcgctctgaacacccctaaggaccacatcggcacccggaatcctgccaacaatgctgccattgtgctgcagctgccacagggcacaacactgcctaagggcttttacgccgagggctctagaggcggctctcaggcctcttccagatcctccagtagatcacgtggtggtagtggcggaagcggcggctccagagtgcagcctaccgagtccatcgtgcggttccccaacatcaccaacctgtgtcctttcggcgaggtgttcaacgctaccagattcgcctctgtgtacgcctggaaccggaagcggatctctaactgcgtggccgactactccgtgctgtacaactctgcctccttcagcaccttcaagtgctacggcgtgtcccctaccaagctgaacgacctgtgcttcaccaacgtgtacgccgactccttcgtgatcaggggcgacgaagttcggcagatcgctcctggacagaccggcaagatcgccgactacaattacaagctgcccgacgacttcaccggctgcgtgatcgcttggaactccaacaacctggactccaaagtcggcggcaactacaactacctgtaccgggccttcagaaagtccaacctgaagcctttcgagcgggacatctccaccgagatctaccaggctggcagcaccccttgcaatggcgttgaaggcgccaactgctacttcccactgcagtcctacggcttccagcctaccaatggcgtgggctaccagccttatagagtggtggtgctgtccttcgagctgctgcatgctcctgctacagtgtgcggccccaagaaatctaccaacctggtcaagaacaag